European Patent Application EP 4 678 745 A1, published January 14, 2026. Title: GUIDE RNA AND METHODS OF USE THEREOF. Applicant: 国立大学法人九州大学. Application WO. The sequence listing filed with the application follows.

SEQUENCE LISTING (182 sequences)

SEQ ID NO: 1 - DNA, 23 bp, Porcine teschovirus-1
  source 1..23: mol_type = genomic DNA
gctgaagcaggctggagacgtgg

SEQ ID NO: 2 - DNA, 9526 bp, synthetic construct
  source 1..9526: mol_type = other DNA
gagggcctatttcccatgattccttcatatttgcatatacgatacaaggctgttagagagataattggaattaatttgactgtaaacacaaagatattagtacaaaatacgtgacgtagaaagtaataatttcttgggtagtttgcagttttaaaattatgttttaaaatggactatcatatgcttaccgtaacttgaaagtatttcgatttcttggctttatatatcttgtggaaaggacgaaacaccgggtcttcgagaagacctgttttagagctagaaatagcaagttaaaataaggctagtccgttatcaacttgaaaaagtggcaccgagtcggtgcttttttgttttagagctagaaatagcaagttaaaataaggctagtccgtttttagcgcgtgcgccaattctgcagacaaatggctctagttattaatagtaatcaattacggggtcattagttcatagcccatatattgagttccgcgttacataacttacggtaaatggcccgcctggctgaccgcccaacgacccccgcccattgacgtcaataatgacgtatgttcccatagtaacgccaatagggactttccattgacgtcaatgggtggagtatttacggtaaactgcccacttggcagtacatcaagtgtatcatatgccaagtacgccccctattgacgtcaatgacggtaaatggcccgcctggcattatgcccagtacatgaccttatgggactttcctacttggcagtacatctacgtattagtcatcgctattaccatggtgatgcggttttggcagtacatcaatgggcgtggatagcggtttgactcacggggatttccaagtctccaccccattgacgtcaatgggagtttgttttggcaccaaaatcaacgggactttccaaaatgtcgtaacaactccgccccattgacgcaaatgggcggtaggcgtgtacggtgggaggtctatataagcagagctggtttagtgaaccgtcagatccgctagagatccgcggccgctaatacgactcactatagggagagccgccaccatgaaacggacagccgacggaagcgagttcgagtcaccaaagaagaagcggaaagtctctgaggtggagttttcccacgagtactggatgagacatgccctgaccctggccaagagggcacgggatgagagggaggtgcctgtgggagccgtgctggtgctgaacaatagagtgatcggcgagggctggaacagagccatcggcctgcacgacccaacagcccatgccgaaattatggccctgagacagggcggcctggtcatgcagaactacagactgattgacgccaccctgtacgtgacattcgagccttgcgtgatgtgcgccggcgccatgatccactctaggatcggccgcgtggtgtttggcgtgaggaactcaaaaagaggcgccgcaggctccctgatgaacgtgctgaactaccccggcatgaatcaccgcgtcgaaattaccgagggaatcctggcagatgaatgtgccgccctgctgtgcgatttctatcggatgcctagacaggtgttcaatgctcagaagaaggcccagagctccatcaactccggaggatctagcggaggctcctctggctctgagacacctggcacaagcgagagcgcaacacctgaaagcagcgggggcagcagcggggggtcagacaagaagtacagcatcggcctggccatcggcaccaactctgtgggctgggccgtgatcaccgacgagtacaaggtgcccagcaagaaattcaaggtgctgggcaacaccgaccggcacagcatcaagaagaacctgatcggagccctgctgttcgacagcggcgaaacagccgaggccacccggctgaagagaaccgccagaagaagatacaccagacggaagaaccggatctgctatctgcaagagatcttcagcaacgagatggccaaggtggacgacagcttcttccacagactggaagagtccttcctggtggaagaggataagaagcacgagcggcaccccatcttcggcaacatcgtggacgaggtggcctaccacgagaagtaccccaccatctaccacctgagaaagaaactggtggacagcaccgacaaggccgacctgcggctgatctatctggccctggcccacatgatcaagttccggggccacttcctgatcgagggcgacctgaaccccgacaacagcgacgtggacaagctgttcatccagctggtgcagacctacaaccagctgttcgaggaaaaccccatcaacgccagcggcgtggacgccaaggccatcctgtctgccagactgagcaagagcagacggctggaaaatctgatcgcccagctgcccggcgagaagaagaatggcctgttcggaaacctgattgccctgagcctgggcctgacccccaacttcaagagcaacttcgacctggccgaggatgccaaactgcagctgagcaaggacacctacgacgacgacctggacaacctgctggcccagatcggcgaccagtacgccgacctgtttctggccgccaagaacctgtccgacgccatcctgctgagcgacatcctgagagtgaacaccgagatcaccaaggcccccctgagcgcctctatgatcaagagatacgacgagcaccaccaggacctgaccctgctgaaagctctcgtgcggcagcagctgcctgagaagtacaaagagattttcttcgaccagagcaagaacggctacgccggctacattgacggcggagccagccaggaagagttctacaagttcatcaagcccatcctggaaaagatggacggcaccgaggaactgctcgtgaagctgaacagagaggacctgctgcggaagcagcggaccttcgacaacggcagcatcccccaccagatccacctgggagagctgcacgccattctgcggcggcaggaagatttttacccattcctgaaggacaaccgggaaaagatcgagaagatcctgaccttccgcatcccctactacgtgggccctctggccaggggaaacagcagattcgcctggatgaccagaaagagcgaggaaaccatcaccccctggaacttcgaggaagtggtggacaagggcgcttccgcccagagcttcatcgagcggatgaccaacttcgataagaacctgcccaacgagaaggtgctgcccaagcacagcctgctgtacgagtacttcaccgtgtataacgagctgaccaaagtgaaatacgtgaccgagggaatgagaaagcccgccttcctgagcggcgagcagaaaaaggccatcgtggacctgctgttcaagaccaaccggaaagtgaccgtgaagcagctgaaagaggactacttcaagaaaatcgagtgcttcgactccgtggaaatctccggcgtggaagatcggttcaacgcctccctgggcacataccacgatctgctgaaaattatcaaggacaaggacttcctggacaatgaggaaaacgaggacattctggaagatatcgtgctgaccctgacactgtttgaggacagagagatgatcgaggaacggctgaaaacctatgcccacctgttcgacgacaaagtgatgaagcagctgaagcggcggagatacaccggctggggcaggctgagccggaagctgatcaacggcatccgggacaagcagtccggcaagacaatcctggatttcctgaagtccgacggcttcgccaacagaaacttcatgcagctgatccacgacgacagcctgacctttaaagaggacatccagaaagcccaggtgtccggccagggcgatagcctgcacgagcacattgccaatctggccggcagccccgccattaagaagggcatcctgcagacagtgaaggtggtggacgagctcgtgaaagtgatgggccggcacaagcccgagaacatcgtgatcgaaatggccagagagaaccagaccacccagaagggacagaagaacagccgcgagagaatgaagcggatcgaagagggcatcaaagagctgggcagccagatcctgaaagaacaccccgtggaaaacacccagctgcagaacgagaagctgtacctgtactacctgcagaatgggcgggatatgtacgtggaccaggaactggacatcaaccggctgtccgactacgatgtggaccatatcgtgcctcagagctttctgaaggacgactccatcgacaacaaggtgctgaccagaagcgacaagaaccggggcaagagcgacaacgtgccctccgaagaggtcgtgaagaagatgaagaactactggcggcagctgctgaacgccaagctgattacccagagaaagttcgacaatctgaccaaggccgagagaggcggcctgagcgaactggataaggccggcttcatcaagagacagctggtggaaacccggcagatcacaaagcacgtggcacagatcctggactcccggatgaacactaagtacgacgagaatgacaagctgatccgggaagtgaaagtgatcaccctgaagtccaagctggtgtccgatttccggaaggatttccagttttacaaagtgcgcgagatcaacaactaccaccacgcccacgacgcctacctgaacgccgtcgtgggaaccgccctgatcaaaaagtaccctaagctggaaagcgagttcgtgtacggcgactacaaggtgtacgacgtgcggaagatgatcgccaagagcgagcaggaaatcggcaaggctaccgccaagtacttcttctacagcaacatcatgaactttttcaagaccgagattaccctggccaacggcgagatccggaagcggcctctgatcgagacaaacggcgaaaccggggagatcgtgtgggataagggccgggattttgccaccgtgcggaaagtgctgagcatgccccaagtgaatatcgtgaaaaagaccgaggtgcagacaggcggcttcagcaaagagtctatcctgcccaagaggaacagcgataagctgatcgccagaaagaaggactgggaccctaagaagtacggcggcttcgacagccccaccgtggcctattctgtgctggtggtggccaaagtggaaaagggcaagtccaagaaactgaagagtgtgaaagagctgctggggatcaccatcatggaaagaagcagcttcgagaagaatcccatcgactttctggaagccaagggctacaaagaagtgaaaaaggacctgatcatcaagctgcctaagtactccctgttcgagctggaaaacggccggaagagaatgctggcctctgccggcgaactgcagaagggaaacgaactggccctgccctccaaatatgtgaacttcctgtacctggccagccactatgagaagctgaagggctcccccgaggataatgagcagaaacagctgtttgtggaacagcacaagcactacctggacgagatcatcgagcagatcagcgagttctccaagagagtgatcctggccgacgctaatctggacaaagtgctgtccgcctacaacaagcaccgggataagcccatcagagagcaggccgagaatatcatccacctgtttaccctgaccaatctgggagcccctgccgccttcaagtactttgacaccaccatcgaccggaagaggtacaccagcaccaaagaggtgctggacgccaccctgatccaccagagcatcaccggcctgtacgagacacggatcgacctgtctcagctgggaggcgacaaaaggccggcggccacgaaaaaggccggccaggcaaaaaagaaaaaggaattcggcagtggagagggcagaggaagtctgctaacatgcggtgacgtcgaggagaatcctggcccaatgaccgagtacaagcccacggtgcgcctcgccacccgcgacgacgtccccagggccgtacgcaccctcgccgccgcgttcgccgactaccccgccacgcgccacaccgtcgatccggaccgccacatcgagcgggtcaccgagctgcaagaactcttcctcacgcgcgtcgggctcgacatcggcaaggtgtgggtcgcggacgacggcgccgcggtggcggtctggaccacgccggagagcgtcgaagcgggggcggtgttcgccgagatcggcccgcgcatggccgagttgagcggttcccggctggccgcgcagcaacagatggaaggcctcctggcgccgcaccggcccaaggagcccgcgtggttcctggccaccgtcggagtctcgcccgaccaccagggcaagggtctgggcagcgccgtcgtgctccccggagtggaggcggccgagcgcgccggggtgcccgccttcctggagacctccgcgccccgcaacctccccttctacgagcggctcggcttcaccgtcaccgccgacgtcgaggtgcccgaaggaccgcgcacctggtgcatgacccgcaagcccggtgcctgagaattctaactagagctcgctgatcagcctcgactgtgccttctagttgccagccatctgttgtttgcccctcccccgtgccttccttgaccctggaaggtgccactcccactgtcctttcctaataaaatgaggaaattgcatcgcattgtctgagtaggtgtcattctattctggggggtggggtggggcaggacagcaagggggaggattgggaagagaatagcaggcatgctggggagcggccgcaggaacccctagtgatggagttggccactccctctctgcgcgctcgctcgctcactgaggccgggcgaccaaaggtcgcccgacgcccgggctttgcccgggcggcctcagtgagcgagcgagcgcgcagctgcctgcaggggcgcctgatgcggtattttctccttacgcatctgtgcggtatttcacaccgcatacgtcaaagcaaccatagtacgcgccctgtagcggcgcattaagcgcggcgggtgtggtggttacgcgcagcgtgaccgctacacttgccagcgccctagcgcccgctcctttcgctttcttcccttcctttctcgccacgttcgccggctttccccgtcaagctctaaatcgggggctccctttagggttccgatttagtgctttacggcacctcgaccccaaaaaacttgatttgggtgatggttcacgtagtgggccatcgccctgatagacggtttttcgccctttgacgttggagtccacgttctttaatagtggactcttgttccaaactggaacaacactcaaccctatctcgggctattcttttgatttataagggattttgccgatttcggcctattggttaaaaaatgagctgatttaacaaaaatttaacgcgaattttaacaaaatattaacgtttacaattttatggtgcactctcagtacaatctgctctgatgccgcatagttaagccagccccgacacccgccaacacccgctgacgcgccctgacgggcttgtctgctcccggcatccgcttacagacaagctgtgaccgtctccgggagctgcatgtgtcagaggttttcaccgtcatcaccgaaacgcgcgagacgaaagggcctcgtgatacgcctatttttataggttaatgtcatgataataatggtttcttagacgtcaggtggcacttttcggggaaatgtgcgcggaacccctatttgtttatttttctaaatacattcaaatatgtatccgctcatgagacaataaccctgataaatgcttcaataatattgaaaaaggaagagtatgagtattcaacatttccgtgtcgcccttattcccttttttgcggcattttgccttcctgtttttgctcacccagaaacgctggtgaaagtaaaagatgctgaagatcagttgggtgcacgagtgggttacatcgaactggatctcaacagcggtaagatccttgagagttttcgccccgaagaacgttttccaatgatgagcacttttaaagttctgctatgtggcgcggtattatcccgtattgacgccgggcaagagcaactcggtcgccgcatacactattctcagaatgacttggttgagtactcaccagtcacagaaaagcatcttacggatggcatgacagtaagagaattatgcagtgctgccataaccatgagtgataacactgcggccaacttacttctgacaacgatcggaggaccgaaggagctaaccgcttttttgcacaacatgggggatcatgtaactcgccttgatcgttgggaaccggagctgaatgaagccataccaaacgacgagcgtgacaccacgatgcctgtagcaatggcaacaacgttgcgcaaactattaactggcgaactacttactctagcttcccggcaacaattaatagactggatggaggcggataaagttgcaggaccacttctgcgctcggcccttccggctggctggtttattgctgataaatctggagccggtgagcgtggaagccgcggtatcattgcagcactggggccagatggtaagccctcccgtatcgtagttatctacacgacggggagtcaggcaactatggatgaacgaaatagacagatcgctgagataggtgcctcactgattaagcattggtaactgtcagaccaagtttactcatatatactttagattgatttaaaacttcatttttaatttaaaaggatctaggtgaagatcctttttgataatctcatgaccaaaatcccttaacgtgagttttcgttccactgagcgtcagaccccgtagaaaagatcaaaggatcttcttgagatcctttttttctgcgcgtaatctgctgcttgcaaacaaaaaaaccaccgctaccagcggtggtttgtttgccggatcaagagctaccaactctttttccgaaggtaactggcttcagcagagcgcagataccaaatactgtccttctagtgtagccgtagttaggccaccacttcaagaactctgtagcaccgcctacatacctcgctctgctaatcctgttaccagtggctgctgccagtggcgataagtcgtgtcttaccgggttggactcaagacgatagttaccggataaggcgcagcggtcgggctgaacggggggttcgtgcacacagcccagcttggagcgaacgacctacaccgaactgagatacctacagcgtgagctatgagaaagcgccacgcttcccgaagggagaaaggcggacaggtatccggtaagcggcagggtcggaacaggagagcgcacgagggagcttccagggggaaacgcctggtatctttatagtcctgtcgggtttcgccacctctgacttgagcgtcgatttttgtgatgctcgtcaggggggcggagcctatggaaaaacgccagcaacgcggcctttttacggttcctggccttttgctggccttttgctcacatgt

SEQ ID NO: 3 - DNA, 8217 bp, synthetic construct
  source 1..8217: mol_type = other DNA
atatgccaagtacgccccctattgacgtcaatgacggtaaatggcccgcctggcattatgcccagtacatgaccttatgggactttcctacttggcagtacatctacgtattagtcatcgctattaccatggtgatgcggttttggcagtacatcaatgggcgtggatagcggtttgactcacggggatttccaagtctccaccccattgacgtcaatgggagtttgttttggcaccaaaatcaacgggactttccaaaatgtcgtaacaactccgccccattgacgcaaatgggcggtaggcgtgtacggtgggaggtctatataagcagagctggtttagtgaaccgtcagatccgctagagatccgcggccgctaatacgactcactatagggagagccgccaccatgaaacggacagccgacggaagcgagttcgagtcaccaaagaagaagcggaaagtctctgaggtggagttttcccacgagtactggatgagacatgccctgaccctggccaagagggcacgggatgagagggaggtgcctgtgggagccgtgctggtgctgaacaatagagtgatcggcgagggctggaacagagccatcggcctgcacgacccaacagcccatgccgaaattatggccctgagacagggcggcctggtcatgcagaactacagactgattgacgccaccctgtacgtgacattcgagccttgcgtgatgtgcgccggcgccatgatccactctaggatcggccgcgtggtgtttggcgtgaggaactcaaaaagaggcgccgcaggctccctgatgaacgtgctgaactaccccggcatgaatcaccgcgtcgaaattaccgagggaatcctggcagatgaatgtgccgccctgctgtgcgatttctatcggatgcctagacaggtgttcaatgctcagaagaaggcccagagctccatcaactccggaggatctagcggaggctcctctggctctgagacacctggcacaagcgagagcgcaacacctgaaagcagcgggggcagcagcggggggtcagacaagaagtacagcatcggcctggccatcggcaccaactctgtgggctgggccgtgatcaccgacgagtacaaggtgcccagcaagaaattcaaggtgctgggcaacaccgaccggcacagcatcaagaagaacctgatcggagccctgctgttcgacagcggcgaaacagccgaggccacccggctgaagagaaccgccagaagaagatacaccagacggaagaaccggatctgctatctgcaagagatcttcagcaacgagatggccaaggtggacgacagcttcttccacagactggaagagtccttcctggtggaagaggataagaagcacgagcggcaccccatcttcggcaacatcgtggacgaggtggcctaccacgagaagtaccccaccatctaccacctgagaaagaaactggtggacagcaccgacaaggccgacctgcggctgatctatctggccctggcccacatgatcaagttccggggccacttcctgatcgagggcgacctgaaccccgacaacagcgacgtggacaagctgttcatccagctggtgcagacctacaaccagctgttcgaggaaaaccccatcaacgccagcggcgtggacgccaaggccatcctgtctgccagactgagcaagagcagacggctggaaaatctgatcgcccagctgcccggcgagaagaagaatggcctgttcggaaacctgattgccctgagcctgggcctgacccccaacttcaagagcaacttcgacctggccgaggatgccaaactgcagctgagcaaggacacctacgacgacgacctggacaacctgctggcccagatcggcgaccagtacgccgacctgtttctggccgccaagaacctgtccgacgccatcctgctgagcgacatcctgagagtgaacaccgagatcaccaaggcccccctgagcgcctctatgatcaagagatacgacgagcaccaccaggacctgaccctgctgaaagctctcgtgcggcagcagctgcctgagaagtacaaagagattttcttcgaccagagcaagaacggctacgccggctacattgacggcggagccagccaggaagagttctacaagttcatcaagcccatcctggaaaagatggacggcaccgaggaactgctcgtgaagctgaacagagaggacctgctgcggaagcagcggaccttcgacaacggcagcatcccccaccagatccacctgggagagctgcacgccattctgcggcggcaggaagatttttacccattcctgaaggacaaccgggaaaagatcgagaagatcctgaccttccgcatcccctactacgtgggccctctggccaggggaaacagcagattcgcctggatgaccagaaagagcgaggaaaccatcaccccctggaacttcgaggaagtggtggacaagggcgcttccgcccagagcttcatcgagcggatgaccaacttcgataagaacctgcccaacgagaaggtgctgcccaagcacagcctgctgtacgagtacttcaccgtgtataacgagctgaccaaagtgaaatacgtgaccgagggaatgagaaagcccgccttcctgagcggcgagcagaaaaaggccatcgtggacctgctgttcaagaccaaccggaaagtgaccgtgaagcagctgaaagaggactacttcaagaaaatcgagtgcttcgactccgtggaaatctccggcgtggaagatcggttcaacgcctccctgggcacataccacgatctgctgaaaattatcaaggacaaggacttcctggacaatgaggaaaacgaggacattctggaagatatcgtgctgaccctgacactgtttgaggacagagagatgatcgaggaacggctgaaaacctatgcccacctgttcgacgacaaagtgatgaagcagctgaagcggcggagatacaccggctggggcaggctgagccggaagctgatcaacggcatccgggacaagcagtccggcaagacaatcctggatttcctgaagtccgacggcttcgccaacagaaacttcatgcagctgatccacgacgacagcctgacctttaaagaggacatccagaaagcccaggtgtccggccagggcgatagcctgcacgagcacattgccaatctggccggcagccccgccattaagaagggcatcctgcagacagtgaaggtggtggacgagctcgtgaaagtgatgggccggcacaagcccgagaacatcgtgatcgaaatggccagagagaaccagaccacccagaagggacagaagaacagccgcgagagaatgaagcggatcgaagagggcatcaaagagctgggcagccagatcctgaaagaacaccccgtggaaaacacccagctgcagaacgagaagctgtacctgtactacctgcagaatgggcgggatatgtacgtggaccaggaactggacatcaaccggctgtccgactacgatgtggaccatatcgtgcctcagagctttctgaaggacgactccatcgacaacaaggtgctgaccagaagcgacaagaaccggggcaagagcgacaacgtgccctccgaagaggtcgtgaagaagatgaagaactactggcggcagctgctgaacgccaagctgattacccagagaaagttcgacaatctgaccaaggccgagagaggcggcctgagcgaactggataaggccggcttcatcaagagacagctggtggaaacccggcagatcacaaagcacgtggcacagatcctggactcccggatgaacactaagtacgacgagaatgacaagctgatccgggaagtgaaagtgatcaccctgaagtccaagctggtgtccgatttccggaaggatttccagttttacaaagtgcgcgagatcaacaactaccaccacgcccacgacgcctacctgaacgccgtcgtgggaaccgccctgatcaaaaagtaccctaagctggaaagcgagttcgtgtacggcgactacaaggtgtacgacgtgcggaagatgatcgccaagagcgagcaggaaatcggcaaggctaccgccaagtacttcttctacagcaacatcatgaactttttcaagaccgagattaccctggccaacggcgagatccggaagcggcctctgatcgagacaaacggcgaaaccggggagatcgtgtgggataagggccgggattttgccaccgtgcggaaagtgctgagcatgccccaagtgaatatcgtgaaaaagaccgaggtgcagacaggcggcttcagcaaagagtctatcctgcccaagaggaacagcgataagctgatcgccagaaagaaggactgggaccctaagaagtacggcggcttcgacagccccaccgtggcctattctgtgctggtggtggccaaagtggaaaagggcaagtccaagaaactgaagagtgtgaaagagctgctggggatcaccatcatggaaagaagcagcttcgagaagaatcccatcgactttctggaagccaagggctacaaagaagtgaaaaaggacctgatcatcaagctgcctaagtactccctgttcgagctggaaaacggccggaagagaatgctggcctctgccggcgaactgcagaagggaaacgaactggccctgccctccaaatatgtgaacttcctgtacctggccagccactatgagaagctgaagggctcccccgaggataatgagcagaaacagctgtttgtggaacagcacaagcactacctggacgagatcatcgagcagatcagcgagttctccaagagagtgatcctggccgacgctaatctggacaaagtgctgtccgcctacaacaagcaccgggataagcccatcagagagcaggccgagaatatcatccacctgtttaccctgaccaatctgggagcccctgccgccttcaagtactttgacaccaccatcgaccggaagaggtacaccagcaccaaagaggtgctggacgccaccctgatccaccagagcatcaccggcctgtacgagacacggatcgacctgtctcagctgggaggtgactctggcggctcaaaaagaaccgccgacggcagcgaattcgagcccaagaagaagaggaaagtctaaccggtcatcatcaccatcaccattgagtttaaacccgctgatcagcctcgactgtgccttctagttgccagccatctgttgtttgcccctcccccgtgccttccttgaccctggaaggtgccactcccactgtcctttcctaataaaatgaggaaattgcatcgcattgtctgagtaggtgtcattctattctggggggtggggtggggcaggacagcaagggggaggattgggaagacaatagcaggcatgctggggatgcggtgggctctatggcttctgaggcggaaagaaccagctggggctcgataccgtcgacctctagctagagcttggcgtaatcatggtcatagctgtttcctgtgtgaaattgttatccgctcacaattccacacaacatacgagccggaagcataaagtgtaaagcctagggtgcctaatgagtgagctaactcacattaattgcgttgcgctcactgcccgctttccagtcgggaaacctgtcgtgccagctgcattaatgaatcggccaacgcgcggggagaggcggtttgcgtattgggcgctcttccgcttcctcgctcactgactcgctgcgctcggtcgttcggctgcggcgagcggtatcagctcactcaaaggcggtaatacggttatccacagaatcaggggataacgcaggaaagaacatgtgagcaaaaggccagcaaaaggccaggaaccgtaaaaaggccgcgttgctggcgtttttccataggctccgcccccctgacgagcatcacaaaaatcgacgctcaagtcagaggtggcgaaacccgacaggactataaagataccaggcgtttccccctggaagctccctcgtgcgctctcctgttccgaccctgccgcttaccggatacctgtccgcctttctcccttcgggaagcgtggcgctttctcatagctcacgctgtaggtatctcagttcggtgtaggtcgttcgctccaagctgggctgtgtgcacgaaccccccgttcagcccgaccgctgcgccttatccggtaactatcgtcttgagtccaacccggtaagacacgacttatcgccactggcagcagccactggtaacaggattagcagagcgaggtatgtaggcggtgctacagagttcttgaagtggtggcctaactacggctacactagaagaacagtatttggtatctgcgctctgctgaagccagttaccttcggaaaaagagttggtagctcttgatccggcaaacaaaccaccgctggtagcggtggtttttttgtttgcaagcagcagattacgcgcagaaaaaaaggatctcaagaagatcctttgatcttttctacggggtctgacactcagtggaacgaaaactcacgttaagggattttggtcatgagattatcaaaaaggatcttcacctagatccttttaaattaaaaatgaagttttaaatcaatctaaagtatatatgagtaaacttggtctgacagttaccaatgcttaatcagtgaggcacctatctcagcgatctgtctatttcgttcatccatagttgcctgactccccgtcgtgtagataactacgatacgggagggcttaccatctggccccagtgctgcaatgataccgcgagacccacgctcaccggctccagatttatcagcaataaaccagccagccggaagggccgagcgcagaagtggtcctgcaactttatccgcctccatccagtctattaattgttgccgggaagctagagtaagtagttcgccagttaatagtttgcgcaacgttgttgccattgctacaggcatcgtggtgtcacgctcgtcgtttggtatggcttcattcagctccggttcccaacgatcaaggcgagttacatgatcccccatgttgtgcaaaaaagcggttagctccttcggtcctccgatcgttgtcagaagtaagttggccgcagtgttatcactcatggttatggcagcactgcataattctcttactgtcatgccatccgtaagatgcttttctgtgactggtgagtactcaaccaagtcattctgagaatagtgtatgcggcgaccgagttgctcttgcccggcgtcaatacgggataataccgcgccacatagcagaactttaaaagtgctcatcattggaaaacgttcttcggggcgaaaactctcaaggatcttaccgctgttgagatccagttcgatgtaacccactcgtgcacccaactgatcttcagcatcttttactttcaccagcgtttctgggtgagcaaaaacaggaaggcaaaatgccgcaaaaaagggaataagggcgacacggaaatgttgaatactcatactcttcctttttcaatattattgaagcatttatcagggttattgtctcatgagcggatacatatttgaatgtatttagaaaaataaacaaataggggttccgcgcacatttccccgaaaagtgccacctgacgtcgacggatcgggagatcgatctcccgatcccctagggtcgactctcagtacaatctgctctgatgccgcatagttaagccagtatctgctccctgcttgtgtgttggaggtcgctgagtagtgcgcgagcaaaatttaagctacaacaaggcaaggcttgaccgacaattgcatgaagaatctgcttagggttaggcgttttgcgctgcttcgcgatgtacgggccagatatacgcgttgacattgattattgactagttattaatagtaatcaattacggggtcattagttcatagcccatatattgagttccgcgttacataacttacggtaaatggcccgcctggctgaccgcccaacgacccccgcccattgacgtcaataatgacgtatgttcccatagtaacgccaatagggactttccattgacgtcaatgggtggagtatttacggtaaactgcccacttggcagtacatcaagtgtatc

SEQ ID NO: 4 - DNA, 9175 bp, synthetic construct
  source 1..9175: mol_type = other DNA
gagggcctatttcccatgattccttcatatttgcatatacgatacaaggctgttagagagataattggaattaatttgactgtaaacacaaagatattagtacaaaatacgtgacgtagaaagtaataatttcttgggtagtttgcagttttaaaattatgttttaaaatggactatcatatgcttaccgtaacttgaaagtatttcgatttcttggctttatatatcttgtggaaaggacgaaacaccgggtcttcgagaagacctgttttagagctagaaatagcaagttaaaataaggctagtccgttatcaacttgaaaaagtggcaccgagtcggtgcttttttgttttagagctagaaatagcaagttaaaataaggctagtccgtttttagcgcgtgcgccaattctgcagacaaatggctctagaggtacccgttacataacttacggtaaatggcccgcctggctgaccgcccaacgacccccgcccattgacgtcaatagtaacgccaatagggactttccattgacgtcaatgggtggagtatttacggtaaactgcccacttggcagtacatcaagtgtatcatatgccaagtacgccccctattgacgtcaatgacggtaaatggcccgcctggcattgtgcccagtacatgaccttatgggactttcctacttggcagtacatctacgtattagtcatcgctattaccatggtcgaggtgagccccacgttctgcttcactctccccatctcccccccctccccacccccaattttgtatttatttattttttaattattttgtgcagcgatgggggcggggggggggggggggcgcgcgccaggcggggcggggcggggcgaggggcggggcggggcgaggcggagaggtgcggcggcagccaatcagagcggcgcgctccgaaagtttccttttatggcgaggcggcggcggcggcggccctataaaaagcgaagcgcgcggcgggcgggagtcgctgcgacgctgccttcgccccgtgccccgctccgccgccgcctcgcgccgcccgccccggctctgactgaccgcgttactcccacaggtgagcgggcgggacggcccttctcctccgggctgtaattagctgagcaagaggtaagggtttaagggatggttggttggtggggtattaatgtttaattacctggagcacctgcctgaaatcactttttttcaggttggaccggtgccaccatggactataaggaccacgacggagactacaaggatcatgatattgattacaaagacgatgacgataagatggccccaaagaagaagcggaaggtcggtatccacggagtcccagcagccgacaagaagtacagcatcggcctggacatcggcaccaactctgtgggctgggccgtgatcaccgacgagtacaaggtgcccagcaagaaattcaaggtgctgggcaacaccgaccggcacagcatcaagaagaacctgatcggagccctgctgttcgacagcggcgaaacagccgaggccacccggctgaagagaaccgccagaagaagatacaccagacggaagaaccggatctgctatctgcaagagatcttcagcaacgagatggccaaggtggacgacagcttcttccacagactggaagagtccttcctggtggaagaggataagaagcacgagcggcaccccatcttcggcaacatcgtggacgaggtggcctaccacgagaagtaccccaccatctaccacctgagaaagaaactggtggacagcaccgacaaggccgacctgcggctgatctatctggccctggcccacatgatcaagttccggggccacttcctgatcgagggcgacctgaaccccgacaacagcgacgtggacaagctgttcatccagctggtgcagacctacaaccagctgttcgaggaaaaccccatcaacgccagcggcgtggacgccaaggccatcctgtctgccagactgagcaagagcagacggctggaaaatctgatcgcccagctgcccggcgagaagaagaatggcctgttcggaaacctgattgccctgagcctgggcctgacccccaacttcaagagcaacttcgacctggccgaggatgccaaactgcagctgagcaaggacacctacgacgacgacctggacaacctgctggcccagatcggcgaccagtacgccgacctgtttctggccgccaagaacctgtccgacgccatcctgctgagcgacatcctgagagtgaacaccgagatcaccaaggcccccctgagcgcctctatgatcaagagatacgacgagcaccaccaggacctgaccctgctgaaagctctcgtgcggcagcagctgcctgagaagtacaaagagattttcttcgaccagagcaagaacggctacgccggctacattgacggcggagccagccaggaagagttctacaagttcatcaagcccatcctggaaaagatggacggcaccgaggaactgctcgtgaagctgaacagagaggacctgctgcggaagcagcggaccttcgacaacggcagcatcccccaccagatccacctgggagagctgcacgccattctgcggcggcaggaagatttttacccattcctgaaggacaaccgggaaaagatcgagaagatcctgaccttccgcatcccctactacgtgggccctctggccaggggaaacagcagattcgcctggatgaccagaaagagcgaggaaaccatcaccccctggaacttcgaggaagtggtggacaagggcgcttccgcccagagcttcatcgagcggatgaccaacttcgataagaacctgcccaacgagaaggtgctgcccaagcacagcctgctgtacgagtacttcaccgtgtataacgagctgaccaaagtgaaatacgtgaccgagggaatgagaaagcccgccttcctgagcggcgagcagaaaaaggccatcgtggacctgctgttcaagaccaaccggaaagtgaccgtgaagcagctgaaagaggactacttcaagaaaatcgagtgcttcgactccgtggaaatctccggcgtggaagatcggttcaacgcctccctgggcacataccacgatctgctgaaaattatcaaggacaaggacttcctggacaatgaggaaaacgaggacattctggaagatatcgtgctgaccctgacactgtttgaggacagagagatgatcgaggaacggctgaaaacctatgcccacctgttcgacgacaaagtgatgaagcagctgaagcggcggagatacaccggctggggcaggctgagccggaagctgatcaacggcatccgggacaagcagtccggcaagacaatcctggatttcctgaagtccgacggcttcgccaacagaaacttcatgcagctgatccacgacgacagcctgacctttaaagaggacatccagaaagcccaggtgtccggccagggcgatagcctgcacgagcacattgccaatctggccggcagccccgccattaagaagggcatcctgcagacagtgaaggtggtggacgagctcgtgaaagtgatgggccggcacaagcccgagaacatcgtgatcgaaatggccagagagaaccagaccacccagaagggacagaagaacagccgcgagagaatgaagcggatcgaagagggcatcaaagagctgggcagccagatcctgaaagaacaccccgtggaaaacacccagctgcagaacgagaagctgtacctgtactacctgcagaatgggcgggatatgtacgtggaccaggaactggacatcaaccggctgtccgactacgatgtggaccatatcgtgcctcagagctttctgaaggacgactccatcgacaacaaggtgctgaccagaagcgacaagaaccggggcaagagcgacaacgtgccctccgaagaggtcgtgaagaagatgaagaactactggcggcagctgctgaacgccaagctgattacccagagaaagttcgacaatctgaccaaggccgagagaggcggcctgagcgaactggataaggccggcttcatcaagagacagctggtggaaacccggcagatcacaaagcacgtggcacagatcctggactcccggatgaacactaagtacgacgagaatgacaagctgatccgggaagtgaaagtgatcaccctgaagtccaagctggtgtccgatttccggaaggatttccagttttacaaagtgcgcgagatcaacaactaccaccacgcccacgacgcctacctgaacgccgtcgtgggaaccgccctgatcaaaaagtaccctaagctggaaagcgagttcgtgtacggcgactacaaggtgtacgacgtgcggaagatgatcgccaagagcgagcaggaaatcggcaaggctaccgccaagtacttcttctacagcaacatcatgaactttttcaagaccgagattaccctggccaacggcgagatccggaagcggcctctgatcgagacaaacggcgaaaccggggagatcgtgtgggataagggccgggattttgccaccgtgcggaaagtgctgagcatgccccaagtgaatatcgtgaaaaagaccgaggtgcagacaggcggcttcagcaaagagtctatcctgcccaagaggaacagcgataagctgatcgccagaaagaaggactgggaccctaagaagtacggcggcttcgacagccccaccgtggcctattctgtgctggtggtggccaaagtggaaaagggcaagtccaagaaactgaagagtgtgaaagagctgctggggatcaccatcatggaaagaagcagcttcgagaagaatcccatcgactttctggaagccaagggctacaaagaagtgaaaaaggacctgatcatcaagctgcctaagtactccctgttcgagctggaaaacggccggaagagaatgctggcctctgccggcgaactgcagaagggaaacgaactggccctgccctccaaatatgtgaacttcctgtacctggccagccactatgagaagctgaagggctcccccgaggataatgagcagaaacagctgtttgtggaacagcacaagcactacctggacgagatcatcgagcagatcagcgagttctccaagagagtgatcctggccgacgctaatctggacaaagtgctgtccgcctacaacaagcaccgggataagcccatcagagagcaggccgagaatatcatccacctgtttaccctgaccaatctgggagcccctgccgccttcaagtactttgacaccaccatcgaccggaagaggtacaccagcaccaaagaggtgctggacgccaccctgatccaccagagcatcaccggcctgtacgagacacggatcgacctgtctcagctgggaggcgacaaaaggccggcggccacgaaaaaggccggccaggcaaaaaagaaaaaggaattcggcagtggagagggcagaggaagtctgctaacatgcggtgacgtcgaggagaatcctggcccaatgaccgagtacaagcccacggtgcgcctcgccacccgcgacgacgtccccagggccgtacgcaccctcgccgccgcgttcgccgactaccccgccacgcgccacaccgtcgatccggaccgccacatcgagcgggtcaccgagctgcaagaactcttcctcacgcgcgtcgggctcgacatcggcaaggtgtgggtcgcggacgacggcgccgcggtggcggtctggaccacgccggagagcgtcgaagcgggggcggtgttcgccgagatcggcccgcgcatggccgagttgagcggttcccggctggccgcgcagcaacagatggaaggcctcctggcgccgcaccggcccaaggagcccgcgtggttcctggccaccgtcggagtctcgcccgaccaccagggcaagggtctgggcagcgccgtcgtgctccccggagtggaggcggccgagcgcgccggggtgcccgccttcctggagacctccgcgccccgcaacctccccttctacgagcggctcggcttcaccgtcaccgccgacgtcgaggtgcccgaaggaccgcgcacctggtgcatgacccgcaagcccggtgcctgagaattctaactagagctcgctgatcagcctcgactgtgccttctagttgccagccatctgttgtttgcccctcccccgtgccttccttgaccctggaaggtgccactcccactgtcctttcctaataaaatgaggaaattgcatcgcattgtctgagtaggtgtcattctattctggggggtggggtggggcaggacagcaagggggaggattgggaagagaatagcaggcatgctggggagcggccgcaggaacccctagtgatggagttggccactccctctctgcgcgctcgctcgctcactgaggccgggcgaccaaaggtcgcccgacgcccgggctttgcccgggcggcctcagtgagcgagcgagcgcgcagctgcctgcaggggcgcctgatgcggtattttctccttacgcatctgtgcggtatttcacaccgcatacgtcaaagcaaccatagtacgcgccctgtagcggcgcattaagcgcggcgggtgtggtggttacgcgcagcgtgaccgctacacttgccagcgccctagcgcccgctcctttcgctttcttcccttcctttctcgccacgttcgccggctttccccgtcaagctctaaatcgggggctccctttagggttccgatttagtgctttacggcacctcgaccccaaaaaacttgatttgggtgatggttcacgtagtgggccatcgccctgatagacggtttttcgccctttgacgttggagtccacgttctttaatagtggactcttgttccaaactggaacaacactcaaccctatctcgggctattcttttgatttataagggattttgccgatttcggcctattggttaaaaaatgagctgatttaacaaaaatttaacgcgaattttaacaaaatattaacgtttacaattttatggtgcactctcagtacaatctgctctgatgccgcatagttaagccagccccgacacccgccaacacccgctgacgcgccctgacgggcttgtctgctcccggcatccgcttacagacaagctgtgaccgtctccgggagctgcatgtgtcagaggttttcaccgtcatcaccgaaacgcgcgagacgaaagggcctcgtgatacgcctatttttataggttaatgtcatgataataatggtttcttagacgtcaggtggcacttttcggggaaatgtgcgcggaacccctatttgtttatttttctaaatacattcaaatatgtatccgctcatgagacaataaccctgataaatgcttcaataatattgaaaaaggaagagtatgagtattcaacatttccgtgtcgcccttattcccttttttgcggcattttgccttcctgtttttgctcacccagaaacgctggtgaaagtaaaagatgctgaagatcagttgggtgcacgagtgggttacatcgaactggatctcaacagcggtaagatccttgagagttttcgccccgaagaacgttttccaatgatgagcacttttaaagttctgctatgtggcgcggtattatcccgtattgacgccgggcaagagcaactcggtcgccgcatacactattctcagaatgacttggttgagtactcaccagtcacagaaaagcatcttacggatggcatgacagtaagagaattatgcagtgctgccataaccatgagtgataacactgcggccaacttacttctgacaacgatcggaggaccgaaggagctaaccgcttttttgcacaacatgggggatcatgtaactcgccttgatcgttgggaaccggagctgaatgaagccataccaaacgacgagcgtgacaccacgatgcctgtagcaatggcaacaacgttgcgcaaactattaactggcgaactacttactctagcttcccggcaacaattaatagactggatggaggcggataaagttgcaggaccacttctgcgctcggcccttccggctggctggtttattgctgataaatctggagccggtgagcgtggaagccgcggtatcattgcagcactggggccagatggtaagccctcccgtatcgtagttatctacacgacggggagtcaggcaactatggatgaacgaaatagacagatcgctgagataggtgcctcactgattaagcattggtaactgtcagaccaagtttactcatatatactttagattgatttaaaacttcatttttaatttaaaaggatctaggtgaagatcctttttgataatctcatgaccaaaatcccttaacgtgagttttcgttccactgagcgtcagaccccgtagaaaagatcaaaggatcttcttgagatcctttttttctgcgcgtaatctgctgcttgcaaacaaaaaaaccaccgctaccagcggtggtttgtttgccggatcaagagctaccaactctttttccgaaggtaactggcttcagcagagcgcagataccaaatactgtccttctagtgtagccgtagttaggccaccacttcaagaactctgtagcaccgcctacatacctcgctctgctaatcctgttaccagtggctgctgccagtggcgataagtcgtgtcttaccgggttggactcaagacgatagttaccggataaggcgcagcggtcgggctgaacggggggttcgtgcacacagcccagcttggagcgaacgacctacaccgaactgagatacctacagcgtgagctatgagaaagcgccacgcttcccgaagggagaaaggcggacaggtatccggtaagcggcagggtcggaacaggagagcgcacgagggagcttccagggggaaacgcctggtatctttatagtcctgtcgggtttcgccacctctgacttgagcgtcgatttttgtgatgctcgtcaggggggcggagcctatggaaaaacgccagcaacgcggcctttttacggttcctggccttttgctggccttttgctcacatgt

SEQ ID NO: 5 - DNA, 28 bp, synthetic construct
  source 1..28: mol_type = other DNA
caccgccaccgggtcttcgagaagacct

SEQ ID NO: 6 - DNA, 28 bp, synthetic construct
  source 1..28: mol_type = other DNA
aaacaggtcttctcgaagacccggtggc

SEQ ID NO: 7 - DNA, 33 bp, synthetic construct
  source 1..33: mol_type = other DNA
caccgcccccccaccgggtcttcgagaagacct

SEQ ID NO: 8 - DNA, 33 bp, synthetic construct
  source 1..33: mol_type = other DNA
aaacaggtcttctcgaagacccggtgggggggc

SEQ ID NO: 9 - DNA, 38 bp, synthetic construct
  source 1..38: mol_type = other DNA
caccgccccccccccccaccgggtcttcgagaagacct

SEQ ID NO: 10 - DNA, 38 bp, synthetic construct
  source 1..38: mol_type = other DNA
aaacaggtcttctcgaagacccggtggggggggggggc

SEQ ID NO: 11 - DNA, 43 bp, synthetic construct
  source 1..43: mol_type = other DNA
caccgcccccccccccccccccaccgggtcttcgagaagacct

SEQ ID NO: 12 - DNA, 43 bp, synthetic construct
  source 1..43: mol_type = other DNA
aaacaggtcttctcgaagacccggtgggggggggggggggggc

SEQ ID NO: 13 - DNA, 48 bp, synthetic construct
  source 1..48: mol_type = other DNA
caccgccccccccccccccccccccccaccgggtcttcgagaagacct

SEQ ID NO: 14 - DNA, 48 bp, synthetic construct
  source 1..48: mol_type = other DNA
aaacaggtcttctcgaagacccggtggggggggggggggggggggggc

SEQ ID NO: 15 - DNA, 53 bp, synthetic construct
  source 1..53: mol_type = other DNA
caccgcccccccccccccccccccccccccccaccgggtcttcgagaagacct

SEQ ID NO: 16 - DNA, 53 bp, synthetic construct
  source 1..53: mol_type = other DNA
aaacaggtcttctcgaagacccggtgggggggggggggggggggggggggggc

SEQ ID NO: 17 - DNA, 24 bp, synthetic construct
  source 1..24: mol_type = other DNA
caccgctgaagcaggctggagacg

SEQ ID NO: 18 - DNA, 24 bp, synthetic construct
  source 1..24: mol_type = other DNA
aaaccgtctccagcctgcttcagc

SEQ ID NO: 19 - DNA, 288 bp, synthetic construct
  source 1..288: mol_type = other DNA
cgactctctgttggtgttcgattacgagggcagtggttctgaagccgctagcctgagctcactgaactcctctgagtcggatcaggaccaggactacgattatctgaacgagtggggcaaccgattcaagaagctggcggacatgtacggcggtggtgaggacgacggtaccggaagcggagctactaacttcagcctgctgaagcaggctggagacgtggaggagaaccctggacctatggtgagcaagggcgaggaggtcatcaaagagttcatgcgcttcaaggt

SEQ ID NO: 20 - DNA, 20 bp, synthetic construct
  source 1..20: mol_type = other DNA
cgactctctgttggtgttcg

SEQ ID NO: 21 - DNA, 20 bp, synthetic construct
  source 1..20: mol_type = other DNA
accttgaagcgcatgaactc

SEQ ID NO: 22 - DNA, 53 bp, synthetic construct
  source 1..53: mol_type = other DNA
acactctttccctacacgacgctcttccgatctcgactctctgttggtgttcg

SEQ ID NO: 23 - DNA, 54 bp, synthetic construct
  source 1..54: mol_type = other DNA
gtgactggagttcagacgtgtgctcttccgatctaccttgaagcgcatgaactc

SEQ ID NO: 24 - DNA, 54 bp, synthetic construct
  source 1..54: mol_type = other DNA
caccgggggggggggggggggggggggggggggggctgaagcaggctggagacg

SEQ ID NO: 25 - DNA, 54 bp, synthetic construct
  source 1..54: mol_type = other DNA
aaaccgtctccagcctgcttcagccccccccccccccccccccccccccccccc

SEQ ID NO: 26 - DNA, 59 bp, synthetic construct
  source 1..59: mol_type = other DNA
caccggggggggggggggggggggggggggggggggggggctgaagcaggctggagacg

SEQ ID NO: 27 - DNA, 59 bp, synthetic construct
  source 1..59: mol_type = other DNA
aaaccgtctccagcctgcttcagcccccccccccccccccccccccccccccccccccc

SEQ ID NO: 28 - DNA, 64 bp, synthetic construct
  source 1..64: mol_type = other DNA
caccgggggggggggggggggggggggggggggggggggggggggctgaagcaggctggagacg

SEQ ID NO: 29 - DNA, 64 bp, synthetic construct
  source 1..64: mol_type = other DNA
aaaccgtctccagcctgcttcagccccccccccccccccccccccccccccccccccccccccc

SEQ ID NO: 30 - DNA, 288 bp, synthetic construct
  source 1..288: mol_type = other DNA
cgactctctgttggtgttcgattacgagggcagtggttctgaagccgctagcctgagctcactgaactcctctgagtcggatcaggaccaggactacgattatctgaacgagtggggcaaccgattcaagaagctggcggacatgtacggcggtggtgaggacgacggtaccggaagcggagctactaacttcagcctgctgaggcaggctggagacgtggaggagaaccctggacctatggtgagcaagggcgaggaggtcatcaaagagttcatgcgcttcaaggt

SEQ ID NO: 31 - DNA, 23 bp, Homo sapiens
  source 1..23: mol_type = genomic DNA
ttgcatagacctgcccactgtgg

SEQ ID NO: 32 - DNA, 55 bp, synthetic construct
  source 1..55: mol_type = other DNA
acactctttccctacacgacgctcttccgatctagatgctgacggggctcctgtt

SEQ ID NO: 33 - DNA, 56 bp, synthetic construct
  source 1..56: mol_type = other DNA
gtgactggagttcagacgtgtgctcttccgatctgacccagcccctgctctgtgta

SEQ ID NO: 34 - DNA, 25 bp, synthetic construct
  source 1..25: mol_type = other DNA
caccgttgcatagacctgcccactg

SEQ ID NO: 35 - DNA, 25 bp, synthetic construct
  source 1..25: mol_type = other DNA
aaaccagtgggcaggtctatgcaac

SEQ ID NO: 36 - DNA, 23 bp, Homo sapiens
  source 1..23: mol_type = genomic DNA
ttgcatatacctgcccactgagg

SEQ ID NO: 37 - DNA, 23 bp, Homo sapiens
  source 1..23: mol_type = genomic DNA
ttacatagacatgcccactgtgg

SEQ ID NO: 38 - DNA, 53 bp, synthetic construct
  source 1..53: mol_type = other DNA
acactctttccctacacgacgctcttccgatcttggggatccaccatctcatg

SEQ ID NO: 39 - DNA, 56 bp, synthetic construct
  source 1..56: mol_type = other DNA
gtgactggagttcagacgtgtgctcttccgatctattggattccttgggggtttct

SEQ ID NO: 40 - DNA, 52 bp, synthetic construct
  source 1..52: mol_type = other DNA
acactctttccctacacgacgctcttccgatcttccaccatcccatcctgtg

SEQ ID NO: 41 - DNA, 59 bp, synthetic construct
  source 1..59: mol_type = other DNA
gtgactggagttcagacgtgtgctcttccgatctaacaaaaagttcaactccacctaag

SEQ ID NO: 42 - DNA, 23 bp, synthetic construct
  source 1..23: mol_type = other DNA
ggctcaccagataaccctgttgg

SEQ ID NO: 43 - DNA, 20 bp, Mus musculus
  source 1..20: mol_type = genomic DNA
agttgctggaaatcctgtgg

SEQ ID NO: 44 - DNA, 20 bp, Mus musculus
  source 1..20: mol_type = genomic DNA
ttcacgctaggcattgtctg

SEQ ID NO: 45 - DNA, 23 bp, synthetic construct
  source 1..23: mol_type = other DNA
actggagcagtaatgcctggtgg

SEQ ID NO: 46 - DNA, 53 bp, synthetic construct
  source 1..53: mol_type = other DNA
acactctttccctacacgacgctcttccgatctcagggaagtaatgccaggtc

SEQ ID NO: 47 - DNA, 54 bp, synthetic construct
  source 1..54: mol_type = other DNA
gtgactggagttcagacgtgtgctcttccgatcttcagctccatccttccactt

SEQ ID NO: 48 - DNA, 25 bp, synthetic construct
  source 1..25: mol_type = other DNA
caccgactggagcagtaatgcctgg

SEQ ID NO: 49 - DNA, 25 bp, synthetic construct
  source 1..25: mol_type = other DNA
aaacccaggcattactgctccagtc

SEQ ID NO: 50 - DNA, 48 bp, synthetic construct
  source 1..48: mol_type = other DNA
caccgcttccccccccccccccccccccactggagcagtaatgcctgg

SEQ ID NO: 51 - DNA, 48 bp, synthetic construct
  source 1..48: mol_type = other DNA
aaacccaggcattactgctccagtggggggggggggggggggggaagc

SEQ ID NO: 52 - DNA, 48 bp, synthetic construct
  source 1..48: mol_type = other DNA
caccgagcccccccccccccccccccccactggagcagtaatgcctgg

SEQ ID NO: 53 - DNA, 48 bp, synthetic construct
  source 1..48: mol_type = other DNA
aaacccaggcattactgctccagtgggggggggggggggggggggctc

SEQ ID NO: 54 - DNA, 48 bp, synthetic construct
  source 1..48: mol_type = other DNA
caccgcggccccccccccccccccccccactggagcagtaatgcctgg

SEQ ID NO: 55 - DNA, 48 bp, synthetic construct
  source 1..48: mol_type = other DNA
aaacccaggcattactgctccagtggggggggggggggggggggccgc

SEQ ID NO: 56 - DNA, 23 bp, Porcine teschovirus-1
  source 1..23: mol_type = genomic DNA
ggagacgtggaggagaaccctgg

SEQ ID NO: 57 - DNA, 24 bp, synthetic construct
  source 1..24: mol_type = other DNA
caccggagacgtggaggagaaccc

SEQ ID NO: 58 - DNA, 24 bp, synthetic construct
  source 1..24: mol_type = other DNA
aaacgggttctcctccacgtctcc

SEQ ID NO: 59 - DNA, 21 bp, synthetic construct
  source 1..21: mol_type = other DNA
caccgacgtggaggagaaccc

SEQ ID NO: 60 - DNA, 21 bp, synthetic construct
  source 1..21: mol_type = other DNA
aaacgggttctcctccacgtc

SEQ ID NO: 61 - DNA, 30 bp, synthetic construct
  source 1..30: mol_type = other DNA
caccgaggctggagacgtggaggagaaccc

SEQ ID NO: 62 - DNA, 30 bp, synthetic construct
  source 1..30: mol_type = other DNA
aaacgggttctcctccacgtctccagcctc

SEQ ID NO: 63 - DNA, 9760 bp, synthetic construct
  source 1..9760: mol_type = other DNA
ttgctggcgtttttccataggctccgcccccctgacgagcatcacaaaaatcgacgctcaagtcagaggtggcgaaacccgacaggactataaagataccaggcgtttccccctggaagctccctcgtgcgctctcctgttccgaccctgccgcttaccggatacctgtccgcctttctcccttcgggaagcgtggcgctttctcatagctcacgctgtaggtatctcagttcggtgtaggtcgttcgctccaagctgggctgtgtgcacgaaccccccgttcagcccgaccgctgcgccttatccggtaactatcgtcttgagtccaacccggtaagacacgacttatcgccactggcagcagccactggtaacaggattagcagagcgaggtatgtaggcggtgctacagagttcttgaagtggtggcctaactacggctacactagaagaacagtatttggtatctgcgctctgctgaagccagttaccttcggaaaaagagttggtagctcttgatccggcaaacaaaccaccgctggtagcggtggtttttttgtttgcaagcagcagattacgcgcagaaaaaaaggatctcaagaagatcctttgatcttttctacggggtctgacgctcagtggaacgaaaactcacgttaagggattttggtcatgagattatcaaaaaggatcttcacctagatccttttaaattaaaaatgaagttttaaatcaatctaaagtatatatgagtaaacttggtctgacagttaccaatgcttaatcagtgaggcacctatctcagcgatctgtctatttcgttcatccatagttgcctgactccccgtcgtgtagataactacgatacgggagggcttaccatctggccccagtgctgcaatgataccgcgagacccacgctcaccggctccagatttatcagcaataaaccagccagccggaagggccgagcgcagaagtggtcctgcaactttatccgcctccatccagtctattaattgttgccgggaagctagagtaagtagttcgccagttaatagtttgcgcaacgttgttgccattgctacaggcatcgtggtgtcacgctcgtcgtttggtatggcttcattcagctccggttcccaacgatcaaggcgagttacatgatcccccatgttgtgcaaaaaagcggttagctccttcggtcctccgatcgttgtcagaagtaagttggccgcagtgttatcactcatggttatggcagcactgcataattctcttactgtcatgccatccgtaagatgcttttctgtgactggtgagtactcaaccaagtcattctgagaatagtgtatgcggcgaccgagttgctcttgcccggcgtcaatacgggataataccgcgccacatagcagaactttaaaagtgctcatcattggaaaacgttcttcggggcgaaaactctcaaggatcttaccgctgttgagatccagttcgatgtaacccactcgtgcacccaactgatcttcagcatcttttactttcaccagcgtttctgggtgagcaaaaacaggaaggcaaaatgccgcaaaaaagggaataagggcgacacggaaatgttgaatactcatactcttcctttttcaatattattgaagcatttatcagggttattgtctcatgagcggatacatatttgaatgtatttagaaaaataaacaaataggggttccgcgcacatttccccgaaaagtgccacctgacgtcgacggatcgggagatcgatctcccgatcccctagggtcgactctcagtacaatctgctctgatgccgcatagttaagccagtatctgctccctgcttgtgtgttggaggtcgctgagtagtgcgcgagcaaaatttaagctacaacaaggcaaggcttgaccgacaattgcatgaagaatctgcttagggttaggcgttttgcgctgcttcgcgatgtacgggccagatatacgcgtggatccctgcagttaattaaagagggcctatttcccatgattccttcatatttgcatatacgatacaaggctgttagagagataattagaattaatttgactgtaaacacaaagatattagtacaaaatacgtgacgtagaaagtaataatttcttgggtagtttgcagttttaaaattatgttttaaaatggactatcatatgcttaccgtaacttgaaagtatttcgatttcttggctttatatatcttgtggaaaggacgaaacaccgggtcttcgagaagacctgttttagagctagaaatagcaagttaaaataaggctagtccgttatcaacttgaaaaagtggcaccgagtcggtgctttttttatgcatggtaccgacattgattattgactagttattaatagtaatcaattacggggtcattagttcatagcccatatatggagttccgcgttacataacttacggtaaatggcccgcctggctgaccgcccaacgacccccgcccattgacgtcaataatgacgtatgttcccatagtaacgccaatagggactttccattgacgtcaatgggtggagtatttacggtaaactgcccacttggcagtacatcaagtgtatcatatgccaagtacgccccctattgacgtcaatgacggtaaatggcccgcctggcattatgcccagtacatgaccttatgggactttcctacttggcagtacatctacgtattagtcatcgctattaccatggtgatgcggttttggcagtacatcaatgggcgtggatagcggtttgactcacggggatttccaagtctccaccccattgacgtcaatgggagtttgttttggcaccaaaatcaacgggactttccaaaatgtcgtaacaactccgccccattgacgcaaatgggcggtaggcgtgtacggtgggaggtctatataagcagagctggtttagtgaaccgtcagatccgctagagatccgcggccgccaccatgaagaggaccgccgatggctctgagttcgagagccccaagaagaagcggaaggtggacagcctgctgatgaaccggagaaagttcctgtatcagtttaagaatgtgaggtgggcaaagggcaggcgcgagacctacctgtgctatgtggtgaagcggagagatagcgccacatctttcagcctggactttggctacctgcggaacaagaatggctgccacgtggagctgctgtttctgagatacatctccgactgggatctggacccaggcaggtgttatcgcgtgacctggttcacatcctggtctccctgctacgattgtgcccggcacgtggccgactttctgagaggcaaccctaatctgtctctgaggatcttcaccgcccgcctgtatttttgcgaggataggaaggccgagccagagggactgaggcgcctgcacagggccggcgtgcagatcgccatcatgacattcaaggactacttttattgttggaacaccttcgtggagaatcacgagcggacatttaaggcctgggagggactgcacgagaactccgtgcggctgtctagacagctgcggagaatcctgctgccaagcggctccgagaccccaggcacatctgagagcgccacccctgagagcgacaagaagtacagcatcggcctggccatcggcaccaactctgtgggctgggccgtgatcaccgacgagtacaaggtgcccagcaagaaattcaaggtgctgggcaacaccgaccggcacagcatcaagaagaacctgatcggagccctgctgttcgacagcggcgaaacagccgaggccacccggctgaagagaaccgccagaagaagatacaccagacggaagaaccggatctgctatctgcaagagatcttcagcaacgagatggccaaggtggacgacagcttcttccacagactggaagagtccttcctggtggaagaggataagaagcacgagcggcaccccatcttcggcaacatcgtggacgaggtggcctaccacgagaagtaccccaccatctaccacctgagaaagaaactggtggacagcaccgacaaggccgacctgcggctgatctatctggccctggcccacatgatcaagttccggggccacttcctgatcgagggcgacctgaaccccgacaacagcgacgtggacaagctgttcatccagctggtgcagacctacaaccagctgttcgaggaaaaccccatcaacgccagcggcgtggacgccaaggccatcctgtctgccagactgagcaagagcagacggctggaaaatctgatcgcccagctgcccggcgagaagaagaatggcctgttcggaaacctgattgccctgagcctgggcctgacccccaacttcaagagcaacttcgacctggccgaggatgccaaactgcagctgagcaaggacacctacgacgacgacctggacaacctgctggcccagatcggcgaccagtacgccgacctgtttctggccgccaagaacctgtccgacgccatcctgctgagcgacatcctgagagtgaacaccgagatcaccaaggcccccctgagcgcctctatgatcaagagatacgacgagcaccaccaggacctgaccctgctgaaagctctcgtgcggcagcagctgcctgagaagtacaaagagattttcttcgaccagagcaagaacggctacgccggctacattgacggcggagccagccaggaagagttctacaagttcatcaagcccatcctggaaaagatggacggcaccgaggaactgctcgtgaagctgaacagagaggacctgctgcggaagcagcggaccttcgacaacggcagcatcccccaccagatccacctgggagagctgcacgccattctgcggcggcaggaagatttttacccattcctgaaggacaaccgggaaaagatcgagaagatcctgaccttccgcatcccctactacgtgggccctctggccaggggaaacagcagattcgcctggatgaccagaaagagcgaggaaaccatcaccccctggaacttcgaggaagtggtggacaagggcgcttccgcccagagcttcatcgagcggatgaccaacttcgataagaacctgcccaacgagaaggtgctgcccaagcacagcctgctgtacgagtacttcaccgtgtataacgagctgaccaaagtgaaatacgtgaccgagggaatgagaaagcccgccttcctgagcggcgagcagaaaaaggccatcgtggacctgctgttcaagaccaaccggaaagtgaccgtgaagcagctgaaagaggactacttcaagaaaatcgagtgcttcgactccgtggaaatctccggcgtggaagatcggttcaacgcctccctgggcacataccacgatctgctgaaaattatcaaggacaaggacttcctggacaatgaggaaaacgaggacattctggaagatatcgtgctgaccctgacactgtttgaggacagagagatgatcgaggaacggctgaaaacctatgcccacctgttcgacgacaaagtgatgaagcagctgaagcggcggagatacaccggctggggcaggctgagccggaagctgatcaacggcatccgggacaagcagtccggcaagacaatcctggatttcctgaagtccgacggcttcgccaacagaaacttcatgcagctgatccacgacgacagcctgacctttaaagaggacatccagaaagcccaggtgtccggccagggcgatagcctgcacgagcacattgccaatctggccggcagccccgccattaagaagggcatcctgcagacagtgaaggtggtggacgagctcgtgaaagtgatgggccggcacaagcccgagaacatcgtgatcgaaatggccagagagaaccagaccacccagaagggacagaagaacagccgcgagagaatgaagcggatcgaagagggcatcaaagagctgggcagccagatcctgaaagaacaccccgtggaaaacacccagctgcagaacgagaagctgtacctgtactacctgcagaatgggcgggatatgtacgtggaccaggaactggacatcaaccggctgtccgactacgatgtggaccatatcgtgcctcagagctttctgaaggacgactccatcgacaacaaggtgctgaccagaagcgacaagaaccggggcaagagcgacaacgtgccctccgaagaggtcgtgaagaagatgaagaactactggcggcagctgctgaacgccaagctgattacccagagaaagttcgacaatctgaccaaggccgagagaggcggcctgagcgaactggataaggccggcttcatcaagagacagctggtggaaacccggcagatcacaaagcacgtggcacagatcctggactcccggatgaacactaagtacgacgagaatgacaagctgatccgggaagtgaaagtgatcaccctgaagtccaagctggtgtccgatttccggaaggatttccagttttacaaagtgcgcgagatcaacaactaccaccacgcccacgacgcctacctgaacgccgtcgtgggaaccgccctgatcaaaaagtaccctaagctggaaagcgagttcgtgtacggcgactacaaggtgtacgacgtgcggaagatgatcgccaagagcgagcaggaaatcggcaaggctaccgccaagtacttcttctacagcaacatcatgaactttttcaagaccgagattaccctggccaacggcgagatccggaagcggcctctgatcgagacaaacggcgaaaccggggagatcgtgtgggataagggccgggattttgccaccgtgcggaaagtgctgagcatgccccaagtgaatatcgtgaaaaagaccgaggtgcagacaggcggcttcagcaaagagtctatcctgcccaagaggaacagcgataagctgatcgccagaaagaaggactgggaccctaagaagtacggcggcttcgacagccccaccgtggcctattctgtgctggtggtggccaaagtggaaaagggcaagtccaagaaactgaagagtgtgaaagagctgctggggatcaccatcatggaaagaagcagcttcgagaagaatcccatcgactttctggaagccaagggctacaaagaagtgaaaaaggacctgatcatcaagctgcctaagtactccctgttcgagctggaaaacggccggaagagaatgctggcctctgccggcgaactgcagaagggaaacgaactggccctgccctccaaatatgtgaacttcctgtacctggccagccactatgagaagctgaagggctcccccgaggataatgagcagaaacagctgtttgtggaacagcacaagcactacctggacgagatcatcgagcagatcagcgagttctccaagagagtgatcctggccgacgctaatctggacaaagtgctgtccgcctacaacaagcaccgggataagcccatcagagagcaggccgagaatatcatccacctgtttaccctgaccaatctgggagcccctgccgccttcaagtactttgacaccaccatcgaccggaagaggtacaccagcaccaaagaggtgctggacgccaccctgatccaccagagcatcaccggcctgtacgagacacggatcgacctgtctcagctgggaggtgacagcggcgggagcggcgggagcggggggagcactaatctgagcgacatcattgagaaggagactgggaaacagctggtcattcaggagtccatcctgatgctgcctgaggaggtggaggaagtgatcggcaacaagccagagtctgacatcctggtgcacaccgcctacgacgagtccacagatgagaatgtgatgctgctgacctctgacgcccccgagtataagccttgggccctggtcatccaggattctaacggcgagaataagatcaagatgctgagcggaggatccggaggatctggaggcagcaccaacctgtctgacatcatcgagaaggagacaggcaagcagctggtcatccaggagagcatcctgatgctgcccgaagaagtcgaagaagtgatcggaaacaagcctgagagcgatatcctggtccataccgcctacgacgagagtaccgacgaaaatgtgatgctgctgacatccgacgccccagagtataagccctgggctctggtcatccaggattccaacggagagaacaaaatcaaaatgctgtctggcggctcaaaaagaaccgccgacggcagcgaattcgagcccaagaagaagaggaaagtcggaagcggagagggcagaggaagtctgctaacatgcggtgacgtcgaggagaatcctggcccaatgaccgagtacaagcccacggtgcgcctcgccacccgcgacgacgtccccagggccgtacgcaccctcgccgccgcgttcgccgactaccccgccacgcgccacaccgtcgatccggaccgccacatcgagcgggtcaccgagctgcaagaactcttcctcacgcgcgtcgggctcgacatcggcaaggtgtgggtcgcggacgacggcgccgcggtggcggtctggaccacgccggagagcgtcgaagcgggggcggtgttcgccgagatcggcccgcgcatggccgagttgagcggttcccggctggccgcgcagcaacagatggaaggcctcctggcgccgcaccggcccaaggagcccgcgtggttcctggccaccgtcggagtctcgcccgaccaccagggcaagggtctgggcagcgccgtcgtgctccccggagtggaggcggccgagcgcgccggggtgcccgccttcctggagacctccgcgccccgcaacctccccttctacgagcggctcggcttcaccgtcaccgccgacgtcgaggtgcccgaaggaccgcgcacctggtgcatgacccgcaagcccggtgcctgagtttaaacccgctgatcagcctcgactgtgccttctagttgccagccatctgttgtttgcccctcccccgtgccttccttgaccctggaaggtgccactcccactgtcctttcctaataaaatgaggaaattgcatcgcattgtctgagtaggtgtcattctattctggggggtggggtggggcaggacagcaagggggaggattgggaagagaatagcaggcatgctggggatgcggtgggctctatggcttctgaggcggaaagaaccagctggggctcgataccgtcgacctctagctagagcttggcgtaatcatggtcatagatgtttcctgtgtgaaattgttatccgctcacaattccacacaacatacgagccggaagcataaagtgtaaagcctagggtgcctaatgagtgagctaactcacattaattgcgttgcgctcactgcccgctttccagtcgggaaacctgtcgtgccagctgcattaatgaatcggccaacgcgcggggagaggcggtttgcgtattgggcgctcttccgcttcctcgctcactgactcgctgcgctcggtcgttcggctgcggcgagcggtatcagctcactcaaaggcggtaatacggttatccacagaatcaggggataacgcaggaaagaacatgtgagcaaaaggccagcaaaaggccaggaaccgtaaaaaggccgcg

SEQ ID NO: 64 - DNA, 9916 bp, synthetic construct
  source 1..9916: mol_type = other DNA
ttgctggcgtttttccataggctccgcccccctgacgagcatcacaaaaatcgacgctcaagtcagaggtggcgaaacccgacaggactataaagataccaggcgtttccccctggaagctccctcgtgcgctctcctgttccgaccctgccgcttaccggatacctgtccgcctttctcccttcgggaagcgtggcgctttctcatagctcacgctgtaggtatctcagttcggtgtaggtcgttcgctccaagctgggctgtgtgcacgaaccccccgttcagcccgaccgctgcgccttatccggtaactatcgtcttgagtccaacccggtaagacacgacttatcgccactggcagcagccactggtaacaggattagcagagcgaggtatgtaggcggtgctacagagttcttgaagtggtggcctaactacggctacactagaagaacagtatttggtatctgcgctctgctgaagccagttaccttcggaaaaagagttggtagctcttgatccggcaaacaaaccaccgctggtagcggtggtttttttgtttgcaagcagcagattacgcgcagaaaaaaaggatctcaagaagatcctttgatcttttctacggggtctgacgctcagtggaacgaaaactcacgttaagggattttggtcatgagattatcaaaaaggatcttcacctagatccttttaaattaaaaatgaagttttaaatcaatctaaagtatatatgagtaaacttggtctgacagttaccaatgcttaatcagtgaggcacctatctcagcgatctgtctatttcgttcatccatagttgcctgactccccgtcgtgtagataactacgatacgggagggcttaccatctggccccagtgctgcaatgataccgcgagacccacgctcaccggctccagatttatcagcaataaaccagccagccggaagggccgagcgcagaagtggtcctgcaactttatccgcctccatccagtctattaattgttgccgggaagctagagtaagtagttcgccagttaatagtttgcgcaacgttgttgccattgctacaggcatcgtggtgtcacgctcgtcgtttggtatggcttcattcagctccggttcccaacgatcaaggcgagttacatgatcccccatgttgtgcaaaaaagcggttagctccttcggtcctccgatcgttgtcagaagtaagttggccgcagtgttatcactcatggttatggcagcactgcataattctcttactgtcatgccatccgtaagatgcttttctgtgactggtgagtactcaaccaagtcattctgagaatagtgtatgcggcgaccgagttgctcttgcccggcgtcaatacgggataataccgcgccacatagcagaactttaaaagtgctcatcattggaaaacgttcttcggggcgaaaactctcaaggatcttaccgctgttgagatccagttcgatgtaacccactcgtgcacccaactgatcttcagcatcttttactttcaccagcgtttctgggtgagcaaaaacaggaaggcaaaatgccgcaaaaaagggaataagggcgacacggaaatgttgaatactcatactcttcctttttcaatattattgaagcatttatcagggttattgtctcatgagcggatacatatttgaatgtatttagaaaaataaacaaataggggttccgcgcacatttccccgaaaagtgccacctgacgtcgacggatcgggagatcgatctcccgatcccctagggtcgactctcagtacaatctgctctgatgccgcatagttaagccagtatctgctccctgcttgtgtgttggaggtcgctgagtagtgcgcgagcaaaatttaagctacaacaaggcaaggcttgaccgacaattgcatgaagaatctgcttagggttaggcgttttgcgctgcttcgcgatgtacgggccagatatacgcgtggatccctgcagttaattaaagagggcctatttcccatgattccttcatatttgcatatacgatacaaggctgttagagagataattagaattaatttgactgtaaacacaaagatattagtacaaaatacgtgacgtagaaagtaataatttcttgggtagtttgcagttttaaaattatgttttaaaatggactatcatatgcttaccgtaacttgaaagtatttcgatttcttggctttatatatcttgtggaaaggacgaaacaccgggtcttcgagaagacctgttttagagctagaaatagcaagttaaaataaggctagtccgttatcaacttgaaaaagtggcaccgagtcggtgctttttttatgcatggtaccgacattgattattgactagttattaatagtaatcaattacggggtcattagttcatagcccatatatggagttccgcgttacataacttacggtaaatggcccgcctggctgaccgcccaacgacccccgcccattgacgtcaataatgacgtatgttcccatagtaacgccaatagggactttccattgacgtcaatgggtggagtatttacggtaaactgcccacttggcagtacatcaagtgtatcatatgccaagtacgccccctattgacgtcaatgacggtaaatggcccgcctggcattatgcccagtacatgaccttatgggactttcctacttggcagtacatctacgtattagtcatcgctattaccatggtgatgcggttttggcagtacatcaatgggcgtggatagcggtttgactcacggggatttccaagtctccaccccattgacgtcaatgggagtttgttttggcaccaaaatcaacgggactttccaaaatgtcgtaacaactccgccccattgacgcaaatgggcggtaggcgtgtacggtgggaggtctatataagcagagctggtttagtgaaccgtcagatccgctagagatccgcggccgccaccatgaagaggaccgccgatggctctgagttcgagagccccaagaagaagcggaaggtggacagcctgctgatgaaccggagaaagttcctgtatcagtttaagaatgtgaggtgggcaaagggcaggcgcgagacctacctgtgctatgtggtgaagcggagagatagcgccacatctttcagcctggactttggctacctgcggaacaagaatggctgccacgtggagctgctgtttctgagatacatctccgactgggatctggacccaggcaggtgttatcgcgtgacctggttcacatcctggtctccctgctacgattgtgcccggcacgtggccgactttctgagaggcaaccctaatctgtctctgaggatcttcaccgcccgcctgtatttttgcgaggataggaaggccgagccagagggactgaggcgcctgcacagggccggcgtgcagatcgccatcatgacattcaaggactacttttattgttggaacaccttcgtggagaatcacgagcggacatttaaggcctgggagggactgcacgagaactccgtgcggctgtctagacagctgcggagaatcctgctgccaagcggctccgagaccccaggcacatctgagagcgccacccctgagagcgacaagaagtacagcatcggcctggccatcggcaccaactctgtgggctgggccgtgatcaccgacgagtacaaggtgcccagcaagaaattcaaggtgctgggcaacaccgaccggcacagcatcaagaagaacctgatcggagccctgctgttcgacagcggcgaaacagccgaggccacccggctgaagagaaccgccagaagaagatacaccagacggaagaaccggatctgctatctgcaagagatcttcagcaacgagatggccaaggtggacgacagcttcttccacagactggaagagtccttcctggtggaagaggataagaagcacgagcggcaccccatcttcggcaacatcgtggacgaggtggcctaccacgagaagtaccccaccatctaccacctgagaaagaaactggtggacagcaccgacaaggccgacctgcggctgatctatctggccctggcccacatgatcaagttccggggccacttcctgatcgagggcgacctgaaccccgacaacagcgacgtggacaagctgttcatccagctggtgcagacctacaaccagctgttcgaggaaaaccccatcaacgccagcggcgtggacgccaaggccatcctgtctgccagactgagcaagagcagacggctggaaaatctgatcgcccagctgcccggcgagaagaagaatggcctgttcggaaacctgattgccctgagcctgggcctgacccccaacttcaagagcaacttcgacctggccgaggatgccaaactgcagctgagcaaggacacctacgacgacgacctggacaacctgctggcccagatcggcgaccagtacgccgacctgtttctggccgccaagaacctgtccgacgccatcctgctgagcgacatcctgagagtgaacaccgagatcaccaaggcccccctgagcgcctctatgatcaagagatacgacgagcaccaccaggacctgaccctgctgaaagctctcgtgcggcagcagctgcctgagaagtacaaagagattttcttcgaccagagcaagaacggctacgccggctacattgacggcggagccagccaggaagagttctacaagttcatcaagcccatcctggaaaagatggacggcaccgaggaactgctcgtgaagctgaacagagaggacctgctgcggaagcagcggaccttcgacaacggcagcatcccccaccagatccacctgggagagctgcacgccattctgcggcggcaggaagatttttacccattcctgaaggacaaccgggaaaagatcgagaagatcctgaccttccgcatcccctactacgtgggccctctggccaggggaaacagcagattcgcctggatgaccagaaagagcgaggaaaccatcaccccctggaacttcgaggaagtggtggacaagggcgcttccgcccagagcttcatcgagcggatgaccaacttcgataagaacctgcccaacgagaaggtgctgcccaagcacagcctgctgtacgagtacttcaccgtgtataacgagctgaccaaagtgaaatacgtgaccgagggaatgagaaagcccgccttcctgagcggcgagcagaaaaaggccatcgtggacctgctgttcaagaccaaccggaaagtgaccgtgaagcagctgaaagaggactacttcaagaaaatcgagtgcttcgactccgtggaaatctccggcgtggaagatcggttcaacgcctccctgggcacataccacgatctgctgaaaattatcaaggacaaggacttcctggacaatgaggaaaacgaggacattctggaagatatcgtgctgaccctgacactgtttgaggacagagagatgatcgaggaacggctgaaaacctatgcccacctgttcgacgacaaagtgatgaagcagctgaagcggcggagatacaccggctggggcaggctgagccggaagctgatcaacggcatccgggacaagcagtccggcaagacaatcctggatttcctgaagtccgacggcttcgccaacagaaacttcatgcagctgatccacgacgacagcctgacctttaaagaggacatccagaaagcccaggtgtccggccagggcgatagcctgcacgagcacattgccaatctggccggcagccccgccattaagaagggcatcctgcagacagtgaaggtggtggacgagctcgtgaaagtgatgggccggcacaagcccgagaacatcgtgatcgaaatggccagagagaaccagaccacccagaagggacagaagaacagccgcgagagaatgaagcggatcgaagagggcatcaaagagctgggcagccagatcctgaaagaacaccccgtggaaaacacccagctgcagaacgagaagctgtacctgtactacctgcagaatgggcgggatatgtacgtggaccaggaactggacatcaaccggctgtccgactacgatgtggaccatatcgtgcctcagagctttctgaaggacgactccatcgacaacaaggtgctgaccagaagcgacaagaaccggggcaagagcgacaacgtgccctccgaagaggtcgtgaagaagatgaagaactactggcggcagctgctgaacgccaagctgattacccagagaaagttcgacaatctgaccaaggccgagagaggcggcctgagcgaactggataaggccggcttcatcaagagacagctggtggaaacccggcagatcacaaagcacgtggcacagatcctggactcccggatgaacactaagtacgacgagaatgacaagctgatccgggaagtgaaagtgatcaccctgaagtccaagctggtgtccgatttccggaaggatttccagttttacaaagtgcgcgagatcaacaactaccaccacgcccacgacgcctacctgaacgccgtcgtgggaaccgccctgatcaaaaagtaccctaagctggaaagcgagttcgtgtacggcgactacaaggtgtacgacgtgcggaagatgatcgccaagagcgagcaggaaatcggcaaggctaccgccaagtacttcttctacagcaacatcatgaactttttcaagaccgagattaccctggccaacggcgagatccggaagcggcctctgatcgagacaaacggcgaaaccggggagatcgtgtgggataagggccgggattttgccaccgtgcggaaagtgctgagcatgccccaagtgaatatcgtgaaaaagaccgaggtgcagacaggcggcttcagcaaagagtctatcctgcccaagaggaacagcgataagctgatcgccagaaagaaggactgggaccctaagaagtacggcggcttcgacagccccaccgtggcctattctgtgctggtggtggccaaagtggaaaagggcaagtccaagaaactgaagagtgtgaaagagctgctggggatcaccatcatggaaagaagcagcttcgagaagaatcccatcgactttctggaagccaagggctacaaagaagtgaaaaaggacctgatcatcaagctgcctaagtactccctgttcgagctggaaaacggccggaagagaatgctggcctctgccggcgaactgcagaagggaaacgaactggccctgccctccaaatatgtgaacttcctgtacctggccagccactatgagaagctgaagggctcccccgaggataatgagcagaaacagctgtttgtggaacagcacaagcactacctggacgagatcatcgagcagatcagcgagttctccaagagagtgatcctggccgacgctaatctggacaaagtgctgtccgcctacaacaagcaccgggataagcccatcagagagcaggccgagaatatcatccacctgtttaccctgaccaatctgggagcccctgccgccttcaagtactttgacaccaccatcgaccggaagaggtacaccagcaccaaagaggtgctggacgccaccctgatccaccagagcatcaccggcctgtacgagacacggatcgacctgtctcagctgggaggtgacagcggcgggagcggcgggagcggggggagcactaatctgagcgacatcattgagaaggagactgggaaacagctggtcattcaggagtccatcctgatgctgcctgaggaggtggaggaagtgatcggcaacaagccagagtctgacatcctggtgcacaccgcctacgacgagtccacagatgagaatgtgatgctgctgacctctgacgcccccgagtataagccttgggccctggtcatccaggattctaacggcgagaataagatcaagatgctgagcggaggatccggaggatctggaggcagcaccaacctgtctgacatcatcgagaaggagacaggcaagcagctggtcatccaggagagcatcctgatgctgcccgaagaagtcgaagaagtgatcggaaacaagcctgagagcgatatcctggtccataccgcctacgacgagagtaccgacgaaaatgtgatgctgctgacatccgacgccccagagtataagccctgggctctggtcatccaggattccaacggagagaacaaaatcaaaatgctgtctggcggctcaaaaagaaccgccgacggcagcgaattcgagcccaagaagaagaggaaagtcggaagcggagctactaacttcagcctgctgaagcaggctggagacgtggaggagaaccctggacctatggtgagcaagggcgaggagctgttcaccggggtggtgcccatcctggtcgagctggacggcgacgtaaacggccacaagttcagcgtgtccggcgagggcgagggcgatgccacctacggcaagctgaccctgaagttcatctgcaccaccggcaagctgcccgtgccctggcccaccctcgtgaccaccctgacctatggagtgcagtgcttcagccgctaccccgaccacatgaagcagcacgacttcttcaagtccgccatgcccgaaggctacgtccaggagcgcaccatcttcttcaaggacgacggcaactacaagacccgcgccgaggtgaagttcgagggcgacaccctggtgaaccgcatcgagctgaagggcatcgacttcaaggaggacggcaacatcctggggcacaagctggagtacaactacaacagccacaacgtctatatcatggccgacaagcagaagaacggcatcaaggtgaacttcaagatccgccacaacatcgaggacggcagcgtgcagctcgccgaccactaccagcagaacacccccatcggcgacggccccgtgctgctgcccgacaaccactacctgagcacccagtccgccctgagcaaagaccccaacgagaagcgcgatcacatggtcctgctggagttcgtgaccgccgccgggatcactctcggcatggacgagctgtacaagtctggtggttctcccaagaagaaaaggaaagtctaagtttaaacccgctgatcagcctcgactgtgccttctagttgccagccatctgttgtttgcccctcccccgtgccttccttgaccctggaaggtgccactcccactgtcctttcctaataaaatgaggaaattgcatcgcattgtctgagtaggtgtcattctattctggggggtggggtggggcaggacagcaagggggaggattgggaagagaatagcaggcatgctggggatgcggtgggctctatggcttctgaggcggaaagaaccagctggggctcgataccgtcgacctctagctagagcttggcgtaatcatggtcatagatgtttcctgtgtgaaattgttatccgctcacaattccacacaacatacgagccggaagcataaagtgtaaagcctagggtgcctaatgagtgagctaactcacattaattgcgttgcgctcactgcccgctttccagtcgggaaacctgtcgtgccagctgcattaatgaatcggccaacgcgcggggagaggcggtttgcgtattgggcgctcttccgcttcctcgctcactgactcgctgcgctcggtcgttcggctgcggcgagcggtatcagctcactcaaaggcggtaatacggttatccacagaatcaggggataacgcaggaaagaacatgtgagcaaaaggccagcaaaaggccaggaaccgtaaaaaggccgcg

SEQ ID NO: 65 - DNA, 701 bp, synthetic construct
  source 1..701: mol_type = other DNA
gaattcgagcccaagaagaagaggaaagtcggaagcggagagggcagaggaagtctgctaacatgcggtgacgtcgaggagaatcctggcccaatgaccgagtacaagcccacggtgcgcctcgccacccgcgacgacgtccccagggccgtacgcaccctcgccgccgcgttcgccgactaccccgccacgcgccacaccgtcgatccggaccgccacatcgagcgggtcaccgagctgcaagaactcttcctcacgcgcgtcgggctcgacatcggcaaggtgtgggtcgcggacgacggcgccgcggtggcggtctggaccacgccggagagcgtcgaagcgggggcggtgttcgccgagatcggcccgcgcatggccgagttgagcggttcccggctggccgcgcagcaacagatggaaggcctcctggcgccgcaccggcccaaggagcccgcgtggttcctggccaccgtcggagtctcgcccgaccaccagggcaagggtctgggcagcgccgtcgtgctccccggagtggaggcggccgagcgcgccggggtgcccgccttcctggagacctccgcgccccgcaacctccccttctacgagcggctcggcttcaccgtcaccgccgacgtcgaggtgcccgaaggaccgcgcacctggtgcatgacccgcaagcccggtgcctgagtttaaac

SEQ ID NO: 66 - DNA, 63 bp, synthetic construct
  source 1..63: mol_type = other DNA
agaattcgagcccaagaagaagaggaaagtcggaagcggagagggcagaggaagtctgctaac

SEQ ID NO: 67 - DNA, 32 bp, synthetic construct
  source 1..32: mol_type = other DNA
tgtttaaactcaggcaccgggcttgcgggtca

SEQ ID NO: 68 - DNA, 34 bp, synthetic construct
  source 1..34: mol_type = other DNA
caccgaagcaggctggagacgtggaggagaaccc

SEQ ID NO: 69 - DNA, 34 bp, synthetic construct
  source 1..34: mol_type = other DNA
aaacgggttctcctccacgtctccagcctgcttc

SEQ ID NO: 70 - DNA, 34 bp, synthetic construct
  source 1..34: mol_type = other DNA
caccgaagcagggaggagacgtggaggagaaccc

SEQ ID NO: 71 - DNA, 34 bp, synthetic construct
  source 1..34: mol_type = other DNA
aaacgggttctcctccacgtctcctccctgcttc

SEQ ID NO: 72 - DNA, 23 bp, synthetic construct
  source 1..23: mol_type = other DNA
ggctcgccagataaccctgttgg

SEQ ID NO: 73 - DNA, 23 bp, synthetic construct
  source 1..23: mol_type = other DNA
actggagcggtaatgcctggtgg

SEQ ID NO: 74 - DNA, 20 bp, synthetic construct
  source 1..20: mol_type = other DNA
ggagacgtggaggagaaccc

SEQ ID NO: 75 - DNA, 17 bp, synthetic construct
  source 1..17: mol_type = other DNA
gacgtggaggagaaccc

SEQ ID NO: 76 - DNA, 25 bp, synthetic construct
  source 1..25: mol_type = other DNA
aggctggagacgtggaggagaaccc

SEQ ID NO: 77 - DNA, 28 bp, synthetic construct
  source 1..28: mol_type = other DNA
aggctggagacgtggaggagaaccctgg

SEQ ID NO: 78 - DNA, 35 bp, synthetic construct
  source 1..35: mol_type = other DNA
ctgaagcaggctggagacgtggaggagaaccctgg

SEQ ID NO: 79 - DNA, 30 bp, synthetic construct
  source 1..30: mol_type = other DNA
gaagcaggctggagacgtggaggagaaccc

SEQ ID NO: 80 - DNA, 30 bp, synthetic construct
  source 1..30: mol_type = other DNA
gaagcagggaggagacgtggaggagaaccc

SEQ ID NO: 81 - DNA, 35 bp, synthetic construct; identical to SEQ ID NO: 78
  source 1..35: mol_type = other DNA

SEQ ID NO: 82 - DNA, 19 bp, synthetic construct
  source 1..19: mol_type = other DNA
cgcggccaacaagaagatg

SEQ ID NO: 83 - DNA, 20 bp, synthetic construct
  source 1..20: mol_type = other DNA
cgacgagtaggatgagaccg

SEQ ID NO: 84 - DNA, 20 bp, synthetic construct
  source 1..20: mol_type = other DNA
tgttgccactggtgctaaag

SEQ ID NO: 85 - DNA, 20 bp, synthetic construct
  source 1..20: mol_type = other DNA
acagcagtcttctccgcttc

SEQ ID NO: 86 - DNA, 20 bp, synthetic construct
  source 1..20: mol_type = other DNA
ctcaaggaaccagggatgaa

SEQ ID NO: 87 - DNA, 20 bp, synthetic construct
  source 1..20: mol_type = other DNA
gctgtaatgagctggcatga

SEQ ID NO: 88 - DNA, 21 bp, synthetic construct
  source 1..21: mol_type = other DNA
actacaccgaggaaatgggct

SEQ ID NO: 89 - DNA, 22 bp, synthetic construct
  source 1..22: mol_type = other DNA
cccacaatgccagttaagaaga

SEQ ID NO: 90 - DNA, 20 bp, synthetic construct
  source 1..20: mol_type = other DNA
gcaccgtcaaggctgagaac

SEQ ID NO: 91 - DNA, 19 bp, synthetic construct
  source 1..19: mol_type = other DNA
tggtgaagacgccagtgga

SEQ ID NO: 92 - DNA, 40 bp, synthetic construct
  source 1..40: mol_type = other DNA
caccgccccccccccccccctaacttcagcctgctgaagc

SEQ ID NO: 93 - DNA, 40 bp, synthetic construct
  source 1..40: mol_type = other DNA
aaacgcttcagcaggctgaagttagggggggggggggggc

SEQ ID NO: 94 - DNA, 39 bp, synthetic construct
  source 1..39: mol_type = other DNA
caccgggggggggggggggtaacttcagcctgctgaagc

SEQ ID NO: 95 - DNA, 39 bp, synthetic construct
  source 1..39: mol_type = other DNA
aaacgcttcagcaggctgaagttaccccccccccccccc

SEQ ID NO: 96 - DNA, 40 bp, synthetic construct
  source 1..40: mol_type = other DNA
caccgaaaaaaaaaaaaaaataacttcagcctgctgaagc

SEQ ID NO: 97 - DNA, 40 bp, synthetic construct
  source 1..40: mol_type = other DNA
aaacgcttcagcaggctgaagttatttttttttttttttc

SEQ ID NO: 98 - DNA, 40 bp, synthetic construct
  source 1..40: mol_type = other DNA
caccgttttttttttttttttaacttcagcctgctgaagc

SEQ ID NO: 99 - DNA, 40 bp, synthetic construct
  source 1..40: mol_type = other DNA
aaacgcttcagcaggctgaagttaaaaaaaaaaaaaaaac

SEQ ID NO: 100 - DNA, 25 bp, synthetic construct
  source 1..25: mol_type = other DNA
caccgtaacttcagcctgctgaagc

SEQ ID NO: 101 - DNA, 25 bp, synthetic construct
  source 1..25: mol_type = other DNA
aaacgcttcagcaggctgaagttac

SEQ ID NO: 102 - DNA, 30 bp, synthetic construct
  source 1..30: mol_type = other DNA
caccgccccctaacttcagcctgctgaagc

SEQ ID NO: 103 - DNA, 30 bp, synthetic construct
  source 1..30: mol_type = other DNA
aaacgcttcagcaggctgaagttagggggc

SEQ ID NO: 104 - DNA, 35 bp, synthetic construct
  source 1..35: mol_type = other DNA
caccgcccccccccctaacttcagcctgctgaagc

SEQ ID NO: 105 - DNA, 35 bp, synthetic construct
  source 1..35: mol_type = other DNA
aaacgcttcagcaggctgaagttaggggggggggc

SEQ ID NO: 106 - DNA, 40 bp, synthetic construct; identical to SEQ ID NO: 92
  source 1..40: mol_type = other DNA

SEQ ID NO: 107 - DNA, 40 bp, synthetic construct; identical to SEQ ID NO: 93
  source 1..40: mol_type = other DNA

SEQ ID NO: 108 - DNA, 45 bp, synthetic construct
  source 1..45: mol_type = other DNA
caccgcccccccccccccccccccctaacttcagcctgctgaagc

SEQ ID NO: 109 - DNA, 45 bp, synthetic construct
  source 1..45: mol_type = other DNA
aaacgcttcagcaggctgaagttaggggggggggggggggggggc

SEQ ID NO: 110 - DNA, 50 bp, synthetic construct
  source 1..50: mol_type = other DNA
caccgccccccccccccccccccccccccctaacttcagcctgctgaagc

SEQ ID NO: 111 - DNA, 50 bp, synthetic construct
  source 1..50: mol_type = other DNA
aaacgcttcagcaggctgaagttagggggggggggggggggggggggggc

SEQ ID NO: 112 - DNA, 55 bp, synthetic construct
  source 1..55: mol_type = other DNA
caccgcccccccccccccccccccccccccccccctaacttcagcctgctgaagc

SEQ ID NO: 113 - DNA, 55 bp, synthetic construct
  source 1..55: mol_type = other DNA
aaacgcttcagcaggctgaagttaggggggggggggggggggggggggggggggc

SEQ ID NO: 114 - DNA, 39 bp, synthetic construct
  source 1..39: mol_type = other DNA
caccgcttcagcaggctgataacttcagcctgctgaagc

SEQ ID NO: 115 - DNA, 39 bp, synthetic construct
  source 1..39: mol_type = other DNA
aaacgcttcagcaggctgaagttatcagcctgctgaagc

SEQ ID NO: 116 - DNA, 39 bp, synthetic construct
  source 1..39: mol_type = other DNA
caccggaagtcgtccgacttaacttcagcctgctgaagc

SEQ ID NO: 117 - DNA, 39 bp, synthetic construct
  source 1..39: mol_type = other DNA
aaacgcttcagcaggctgaagttaagtcggacgacttcc

SEQ ID NO: 118 - DNA, 23 bp, synthetic construct
  source 1..23: mol_type = other DNA
ctcgcttcggcagcacatatact

SEQ ID NO: 119 - DNA, 22 bp, synthetic construct
  source 1..22: mol_type = other DNA
acgcttcacgaatttgcgtgtc

SEQ ID NO: 120 - DNA, 43 bp, synthetic construct
  source 1..43: mol_type = other DNA
cttcgatgtcgactcgagtcaaaaagcaccgactcggtgccac

SEQ ID NO: 121 - DNA, 27 bp, synthetic construct
  source 1..27: mol_type = other DNA
gttttagagctagaaatagcaagttaa

SEQ ID NO: 122 - DNA, 20 bp, synthetic construct
  source 1..20: mol_type = other DNA
aagcaccgactcggtgccac

SEQ ID NO: 123 - DNA, 25 bp, synthetic construct
  source 1..25: mol_type = other DNA
caccgcgggagaaaggaacgggagg

SEQ ID NO: 124 - DNA, 25 bp, synthetic construct
  source 1..25: mol_type = other DNA
aaaccctcccgttcctttctcccgc

SEQ ID NO: 125 - DNA, 26 bp, synthetic construct
  source 1..26: mol_type = other DNA
caccgccgggagaaaggaacgggagg

SEQ ID NO: 126 - DNA, 26 bp, synthetic construct
  source 1..26: mol_type = other DNA
aaaccctcccgttcctttctcccggc

SEQ ID NO: 127 - DNA, 27 bp, synthetic construct
  source 1..27: mol_type = other DNA
caccgcccgggagaaaggaacgggagg

SEQ ID NO: 128 - DNA, 27 bp, synthetic construct
  source 1..27: mol_type = other DNA
aaaccctcccgttcctttctcccgggc

SEQ ID NO: 129 - DNA, 28 bp, synthetic construct
  source 1..28: mol_type = other DNA
caccgccccgggagaaaggaacgggagg

SEQ ID NO: 130 - DNA, 28 bp, synthetic construct
  source 1..28: mol_type = other DNA
aaaccctcccgttcctttctcccggggc

SEQ ID NO: 131 - DNA, 29 bp, synthetic construct
  source 1..29: mol_type = other DNA
caccgcccccgggagaaaggaacgggagg

SEQ ID NO: 132 - DNA, 29 bp, synthetic construct
  source 1..29: mol_type = other DNA
aaaccctcccgttcctttctcccgggggc

SEQ ID NO: 133 - DNA, 30 bp, synthetic construct
  source 1..30: mol_type = other DNA
caccgccccccgggagaaaggaacgggagg

SEQ ID NO: 134 - DNA, 30 bp, synthetic construct
  source 1..30: mol_type = other DNA
aaaccctcccgttcctttctcccggggggc

SEQ ID NO: 135 - DNA, 31 bp, synthetic construct
  source 1..31: mol_type = other DNA
caccgcccccccgggagaaaggaacgggagg

SEQ ID NO: 136 - DNA, 31 bp, synthetic construct
  source 1..31: mol_type = other DNA
aaaccctcccgttcctttctcccgggggggc

SEQ ID NO: 137 - DNA, 35 bp, synthetic construct
  source 1..35: mol_type = other DNA
caccgcccccccccccgggagaaaggaacgggagg

SEQ ID NO: 138 - DNA, 35 bp, synthetic construct
  source 1..35: mol_type = other DNA
aaaccctcccgttcctttctcccgggggggggggc

SEQ ID NO: 139 - DNA, 25 bp, synthetic construct
  source 1..25: mol_type = other DNA
caccgccttggtgaagtctcctttg

SEQ ID NO: 140 - DNA, 25 bp, synthetic construct
  source 1..25: mol_type = other DNA
aaaccaaaggagacttcaccaaggc

SEQ ID NO: 141 - DNA, 25 bp, synthetic construct
  source 1..25: mol_type = other DNA
caccggctcgctgagacttcctgga

SEQ ID NO: 142 - DNA, 25 bp, synthetic construct
  source 1..25: mol_type = other DNA
aaactccaggaagtctcagcgagcc

SEQ ID NO: 143 - DNA, 26 bp, synthetic construct
  source 1..26: mol_type = other DNA
caccgcgctcgctgagacttcctgga

SEQ ID NO: 144 - DNA, 26 bp, synthetic construct
  source 1..26: mol_type = other DNA
aaactccaggaagtctcagcgagcgc

SEQ ID NO: 145 - DNA, 27 bp, synthetic construct
  source 1..27: mol_type = other DNA
caccgccgctcgctgagacttcctgga

SEQ ID NO: 146 - DNA, 27 bp, synthetic construct
  source 1..27: mol_type = other DNA
aaactccaggaagtctcagcgagcggc

SEQ ID NO: 147 - DNA, 28 bp, synthetic construct
  source 1..28: mol_type = other DNA
caccgcccgctcgctgagacttcctgga

SEQ ID NO: 148 - DNA, 28 bp, synthetic construct
  source 1..28: mol_type = other DNA
aaactccaggaagtctcagcgagcgggc

SEQ ID NO: 149 - DNA, 29 bp, synthetic construct
  source 1..29: mol_type = other DNA
caccgccccgctcgctgagacttcctgga

SEQ ID NO: 150 - DNA, 29 bp, synthetic construct
  source 1..29: mol_type = other DNA
aaactccaggaagtctcagcgagcggggc

SEQ ID NO: 151 - DNA, 30 bp, synthetic construct
  source 1..30: mol_type = other DNA
caccgcccccgctcgctgagacttcctgga

SEQ ID NO: 152 - DNA, 30 bp, synthetic construct
  source 1..30: mol_type = other DNA
aaactccaggaagtctcagcgagcgggggc

SEQ ID NO: 153 - DNA, 31 bp, synthetic construct
  source 1..31: mol_type = other DNA
caccgccccccgctcgctgagacttcctgga

SEQ ID NO: 154 - DNA, 31 bp, synthetic construct
  source 1..31: mol_type = other DNA
aaactccaggaagtctcagcgagcggggggc

SEQ ID NO: 155 - DNA, 32 bp, synthetic construct
  source 1..32: mol_type = other DNA
caccgcccccccgctcgctgagacttcctgga

SEQ ID NO: 156 - DNA, 32 bp, synthetic construct
  source 1..32: mol_type = other DNA
aaactccaggaagtctcagcgagcgggggggc

SEQ ID NO: 157 - DNA, 26 bp, synthetic construct
  source 1..26: mol_type = other DNA
caccgcaggtagcaaagtgacgccga

SEQ ID NO: 158 - DNA, 26 bp, synthetic construct
  source 1..26: mol_type = other DNA
aaactcggcgtcactttgctacctgc

SEQ ID NO: 159 - DNA, 869 bp, synthetic construct
  source 1..869: mol_type = other DNA
gctagccgcgccgacgcgctggacgatttcgatctcgacatgctgggttctgatgccctcgatgactttgacctggatatgttgggaagcgacgcattggatgactttgatctggacatgctcggctccgatgctctggacgatttcgatctcgatatgttaatcggtaccgagggcagaggaagtcttctaacatgcggtgacgtggaggagaatcccggccctatgaccgagtacaagcccacggtgcgcctcgccacccgcgacgacgtccccagggccgtacgcaccctcgccgccgcgttcgccgactaccccgccacgcgccacaccgtcgatccggaccgccacatcgagcgggtcaccgagctgcaagaactcttcctcacgcgcgtcgggctcgacatcggcaaggtgtgggtcgcggacgacggcgccgcggtggcggtctggaccacgccggagagcgtcgaagcgggggcggtgttcgccgagatcggcccgcgcatggccgagttgagcggttcccggctggccgcgcagcaacagatggaaggcctcctggcgccgcaccggcccaaggagcccgcgtggttcctggccaccgtcggcgtgtcgcccgaccaccagggcaagggtctgggcagcgccgtcgtgctccccggagtggaggcggccgagcgcgccggggtgcccgccttcctggagacctccgcgccccgcaacctccccttctacgagcggctcggcttcaccgtcaccgccgacgtcgaggtgcccgaaggaccgcgcacctggtgcatgacccgcaagcccggtgcctgaccagcacactggcggccgttactagcttctgcagcacgaccggt

SEQ ID NO: 160 - DNA, 363 bp, synthetic construct
  source 1..363: mol_type = other DNA
acatgtgagggcctatttcccatgattccttcatatttgcatatacgatacaaggctgttagagagataattggaattaatttgactgtaaacacaaagatattagtacaaaatacgtgacgtagaaagtaataatttcttgggtagtttgcagttttaaaattatgttttaaaatggactatcatatgcttaccgtaacttgaaagtatttcgatttcttggctttatatatcttgtggaaaggacgaaacaccgggtcttcgagaagacctttttttgttttagagctagaaatagcaagttaaaataaggctagtccgtttttagcgcgtgcgccaattctgcagacaaatggctctaga

SEQ ID NO: 161 - DNA, 55 bp, synthetic construct
  source 1..55: mol_type = other DNA
caccgtaatttctactcttgtagatgtctactaaaacaagccggggttttatttt

SEQ ID NO: 162 - DNA, 55 bp, synthetic construct
  source 1..55: mol_type = other DNA
aaacaaaataaaaccccggcttgttttagtagacatctacaagagtagaaattac

SEQ ID NO: 163 - DNA, 60 bp, synthetic construct
  source 1..60: mol_type = other DNA
caccgccccctaatttctactcttgtagatgtctactaaaacaagccggggttttatttt

SEQ ID NO: 164 - DNA, 60 bp, synthetic construct
  source 1..60: mol_type = other DNA
aaacaaaataaaaccccggcttgttttagtagacatctacaagagtagaaattagggggc

SEQ ID NO: 165 - DNA, 65 bp, synthetic construct
  source 1..65: mol_type = other DNA
caccgcccccccccctaatttctactcttgtagatgtctactaaaacaagccggggttttatttt

SEQ ID NO: 166 - DNA, 65 bp, synthetic construct
  source 1..65: mol_type = other DNA
aaacaaaataaaaccccggcttgttttagtagacatctacaagagtagaaattaggggggggggc

SEQ ID NO: 167 - DNA, 70 bp, synthetic construct
  source 1..70: mol_type = other DNA
caccgccccccccccccccctaatttctactcttgtagatgtctactaaaacaagccggggttttatttt

SEQ ID NO: 168 - DNA, 70 bp, synthetic construct
  source 1..70: mol_type = other DNA
aaacaaaataaaaccccggcttgttttagtagacatctacaagagtagaaattagggggggggggggggc

SEQ ID NO: 169 - DNA, 75 bp, synthetic construct
  source 1..75: mol_type = other DNA
caccgcccccccccccccccccccctaatttctactcttgtagatgtctactaaaacaagccggggttttatttt

SEQ ID NO: 170 - DNA, 75 bp, synthetic construct
  source 1..75: mol_type = other DNA
aaacaaaataaaaccccggcttgttttagtagacatctacaagagtagaaattaggggggggggggggggggggc

SEQ ID NO: 171 - DNA, 80 bp, synthetic construct
  source 1..80: mol_type = other DNA
caccgtaatttctactcttgtagatgtctactaaaacaagccggggcccccccccccccccccccccccccttttatttt

SEQ ID NO: 172 - DNA, 80 bp, synthetic construct
  source 1..80: mol_type = other DNA
aaacaaaataaaagggggggggggggggggggggggggccccggcttgttttagtagacatctacaagagtagaaattac

SEQ ID NO: 173 - DNA, 85 bp, synthetic construct
  source 1..85: mol_type = other DNA
caccgcccccccccccccccccccccccccccccctaatttctactcttgtagatgtctactaaaacaagccggggttttatttt

SEQ ID NO: 174 - DNA, 85 bp, synthetic construct
  source 1..85: mol_type = other DNA
aaacaaaataaaaccccggcttgttttagtagacatctacaagagtagaaattaggggggggggggggggggggggggggggggc

SEQ ID NO: 175 - DNA, 65 bp, synthetic construct
  source 1..65: mol_type = other DNA
caccgtaatttctactcttgtagatccccccccccgtctactaaaacaagccggggttttatttt

SEQ ID NO: 176 - DNA, 65 bp, synthetic construct
  source 1..65: mol_type = other DNA
aaacaaaataaaaccccggcttgttttagtagacggggggggggatctacaagagtagaaattac

SEQ ID NO: 177 - DNA, 80 bp, synthetic construct
  source 1..80: mol_type = other DNA
caccgtaatttctactcttgtagatcccccccccccccccccccccccccgtctactaaaacaagccggggttttatttt

SEQ ID NO: 178 - DNA, 80 bp, synthetic construct
  source 1..80: mol_type = other DNA
aaacaaaataaaaccccggcttgttttagtagacgggggggggggggggggggggggggatctacaagagtagaaattac

SEQ ID NO: 179 - DNA, 65 bp, synthetic construct
  source 1..65: mol_type = other DNA
caccgtaatttctactcttgtagatgtctactaaaacaagccggggccccccccccttttatttt

SEQ ID NO: 180 - DNA, 65 bp, synthetic construct
  source 1..65: mol_type = other DNA
aaacaaaataaaaggggggggggccccggcttgttttagtagacatctacaagagtagaaattac

SEQ ID NO: 181 - DNA, 80 bp, synthetic construct; identical to SEQ ID NO: 171
  source 1..80: mol_type = other DNA

SEQ ID NO: 182 - DNA, 80 bp, synthetic construct; identical to SEQ ID NO: 172
  source 1..80: mol_type = other DNA